European Patent Application EP 4 710 940 A2, published March 18, 2026. Title: METHODS AND COMPOSITIONS FOR PROGRAMMING T CELL DIFFERENTIATION AND ENHANCING T CELL PROLIFERATION. Applicant: THE TRUSTEES OF THE UNIVERSITY OF PENNSYLVANIA. Application EP. The sequence listing filed with the application follows.

SEQUENCE LISTING (40 sequences)

SEQ ID NO: 1-2 - skipped (2 entries)

SEQ ID NO: 3 - DNA, 264 bp, synthetic construct
  misc_feature 1..264: note = Synthetic Construct
  source 1..264: mol_type = other DNA
ggtggctttaccaacagtaccggaatgcccccgggctggaagtcgagcttccattatataccctctaactagtacgccttctgtatgaaacagtttttcctccacgccttctgtatgaaacagtttttcctccacgccttctgtatgaaacagtttttcctccacgccttctgtatgaaacagtttttcctccacgccttctgtatgaaacagtttttcctccacgccttctgtatgaaacagtttttcctccaacagtaccgg

SEQ ID NO: 4 - DNA, 4908 bp, synthetic construct
  misc_feature 1..4908: note = pASP73 (iFOX01-3A + Her2 CAR)
  source 1..4908: mol_type = other DNA
ttagccggaaacccagctgtgtgtggtggttttcacgctgtgagggaagctctggttgggcagcacgttatcgaagttgaagtccagggtatcgccgtccatcaggtcgttgcggatgatggattccatgtcgcagtccagtctctcgatgaacatgccgtccagatcagagggcagcttctcttggtgcagcaggcccattctgccgtagccattacagctggacacgctggagtagccgccgagggcagacatctgcataggatgaggcagtgggacctgcacaggggttttcacttgggtcagccggttcatgccgctggtatgaggcatggtggacacggtgtgaggcagaggtctgccattaacggcgcttgtctgctgggcatgtccagggtgtgtgtggctgctggggttcatcatcttgttgtggctggcctgagagccgtatgtgctcatcacgctattggggcccatcatcacgttctggcccagcactctactattaggctgggccacgccagggtccacaggtgtcatgatgtcgttgtgaggagggctgtcagaggtcagcagctctttcagcagtccaggggcacaattgtactggctcatgccgccgtaggaggacttgttgtcctgcagggtctgaatgggcatctgtggcagagggctcatgctgctctggccgtaggtgtacttctggtagttaggagatgggctgttcaggcttgtgttaggaggggcgaagctgtagcaaggggtctgctgcatcatggtgccggggctgctttgtgtagacacggtcaggctggtagggctgctcagcagattcaggttgtccagcaggttttccatgttctcggggttgctgatctcgctcaggcttggcagtgtgctggccattttggcggcgcttggaggatacaccatgctgtgcacgtcgccttctccgagatcatcctgctcggtcatgatggggctcagtctgccagagatggtgctggcattggcgctggttctgggtctgaaggtggaccagttgtcgaagtcgtcgttgctgtgagagccaggagaggcgggccacttagaaaactggctgccaggagaatcgccagcgccttcttgtccagactgcagagaggccttcttcttggcggctctgcttctgctcttggcgaacttggagttgttgtccatggcagcggcccttctacgaggagacttgccgctcttgccgccttcgggattcagcatccaccaagaggacttgccggtgccttcattctgcacccggatgaacttgctgtgcagggacagattgtgccggatgctgttcttccagccggcggagctattgctgtcgcccttgtccttgaagtagggcacgctcttgaccatccactcgtagatctggctcagggtcagtctcttctcggcgctgctctcaatggccttggtgatcaggtcggcgtagctcagattgccccaggcgtttcttctgctggagctgctctttctaggctgtccagcaagtggtccagcggcagctggaggaacaggaggatgctgagacagaggtccaggtggaggtggttgaggtggagcagggtgcagacatccggcctcaggtccctgaaaatcgccgcaaagtccacctgtagcagcagctgcggctgcggcggcaacagctgcagccacagatccaggagcctgagggaagtcctcgctctcttccagcaggctcaggttgctcatgaagtcggcggacactgcagcagcagaggcagaaggcagtccagcagcagcatcaggattagcggcggcagatccgctaggagcagggctagatgtggcgctgttgctctggctgaactcaggtctaggcagaggccaagcacaagatctaggccgaggcaggggctcgaaatcagggtcgatttccaccacctggggagcctcggccatggtggctttaccaacagtaccggaatgcccccgggctggaagtcgagcttccattatataccctctaactagtacgccttctgtatgaaacagtttttcctccacgccttctgtatgaaacagtttttcctccacgccttctgtatgaaacagtttttcctccacgccttctgtatgaaacagtttttcctccacgccttctgtatgaaacagtttttcctccacgccttctgtatgaaacagtttttcctccaacagtaccggatgcatcgtgaggctccggtgcccgtcagtgggcagagcgcacatcgcccacagtccccgagaagttggggggaggggtcggcaattgaaccggtgcctagagaaggtggcgcggggtaaactgggaaagtgatgtcgtgtactggctccgcctttttcccgagggtgggggagaaccgtatataagtgcagtagtcgccgtgaacgttctttttcgcaacgggtttgccgccagaacacaggtaagtgccgtgtgtggttcccgcgggcctggcctctttacgggttatggcccttgcgtgccttgaattacttccacctggctgcagtacgtgattcttgatcccgagcttcgggttggaagtgggtgggagagttcgaggccttgcgcttaaggagccccttcgcctcgtgcttgagttgaggcctggcctgggcgctggggccgccgcgtgcgaatctggtggcaccttcgcgcctgtctcgctgctttcgataagtctctagccatttaaaatttttgatgacctgctgcgacgctttttttctggcaagatagtcttgtaaatgcgggccaagatctgcacactggtatttcggtttttggggccgcgggcggcgacggggcccgtgcgtcccagcgcacatgttcggcgaggcggggcctgcgagcgcggccaccgagaatcggacgggggtagtctcaagctggccggcctgctctggtgcctggcctcgcgccgccgtgtatcgccccgccctgggcggcaaggctggcccggtcggcaccagttgcgtgagcggaaagatggccgcttcccggccctgctgcagggagctcaaaatggaggacgcggcgctcgggagagcgggcgggtgagtcacccacacaaaggaaaagggcctttccgtcctcagccgtcgcttcatgtgactccactgagtaccgggcgccgtccaggcacctcgattagttctcgtgcttttggagtacgtcgtctttaggttggggggaggggttttatgcgatggagtttccccacactgagtgggtggagactgaagttaggccagcttggcacttgatgtaattctccttggaatttgccctttttgagtttggatcttggttcattctcaagcctcagacagtggttcaaagtttttttcttccatttcaggtgtcgtgattctagagccaccatggccttaccagtgaccgccttgctcctgccgctggccttgctgctccacgccgccaggccggacattcaaatgacacagagtccctcatccctcagtgccagcgtgggcgatcgggtgactataacctgcagagcttctcaggacgtgaataccgctgtggcgtggtaccagcagaagccaggcaaagcgcctaagcttctcatttatagtgccagcttcctgtactcaggtgttccgtctcgcttttctggaagtagaagtgggaccgatttcacattgacgatcagcagcttgcagcccgaagatttcgccacctactactgtcagcagcactacactaccccaccgacatttggtcaaggcacaaaagtagagattaaacgcactggttccaccagcgggagcgggaaacccggctctggggaggggagcgaggtccagctggtggaatccgggggtggtcttgtgcagccaggaggatccttgaggttgtcctgcgccgcaagcggctttaacatcaaagatacatacatccattgggtccgacaggcccctggaaagggcctggagtgggtcgcccggatctacccaactaacgggtacactcgctacgctgatagcgtcaagggtcggtttactatttctgccgacacctcaaaaaacacagcctacctccagatgaactctctcagagctgaggatacagccgtgtactattgcagccggtggggaggcgacgggttctacgctatggatgtgtgggggcagggcacactggtcaccgtgagctcatccggaaccacgacgccagcgccgcgaccaccaacaccggcgcccaccatcgcgtcgcagcccctgtccctgcgcccagaggcgtgccggccagcggcggggggcgcagtgcacacgagggggctggacttcgcctgtgatatctacatctgggcgcccttggccgggacttgtggggtccttctcctgtcactggttatcaccctttactgcaaacggggcagaaagaaactcctgtatatattcaaacaaccatttatgagaccagtacaaactactcaagaggaagatggctgtagctgccgatttccagaagaagaagaaggaggatgtgaactgagagtgaagttcagcaggagcgcagacgcccccgcgtacaagcagggccagaaccagctctataacgagctcaatctaggacgaagagaggagtacgatgttttggacaagagacgtggccgggaccctgagatggggggaaagccgagaaggaagaaccctcaggaaggcctgtacaatgaactgcagaaagataagatggcggaggcctacagtgagattgggatgaaaggcgagcgccggaggggcaaggggcacgatggcctttaccagggtctcagtacagccaccaaggacacctacgacgcccttcacatgcaggccctgccccctcgctaa

SEQ ID NO: 5 - DNA, 180 bp, synthetic construct
  misc_feature 1..180: note = Synthetic NFAT promoter
  source 1..180: mol_type = other DNA
ggaggaaaaactgtttcatacagaaggcgtggaggaaaaactgtttcatacagaaggcgtggaggaaaaactgtttcatacagaaggcgtggaggaaaaactgtttcatacagaaggcgtggaggaaaaactgtttcatacagaaggcgtggaggaaaaactgtttcatacagaaggcgt

SEQ ID NO: 6 - DNA, 32 bp, synthetic construct
  misc_feature 1..32: note = Minimal promoter
  source 1..32: mol_type = other DNA
tagagggtatataatggaagctcgacttccag

SEQ ID NO: 7 - DNA, 1184 bp, synthetic construct
  misc_feature 1..1184: note = EF1alpha promoter
  source 1..1184: mol_type = other DNA
cgtgaggctccggtgcccgtcagtgggcagagcgcacatcgcccacagtccccgagaagttggggggaggggtcggcaattgaaccggtgcctagagaaggtggcgcggggtaaactgggaaagtgatgtcgtgtactggctccgcctttttcccgagggtgggggagaaccgtatataagtgcagtagtcgccgtgaacgttctttttcgcaacgggtttgccgccagaacacaggtaagtgccgtgtgtggttcccgcgggcctggcctctttacgggttatggcccttgcgtgccttgaattacttccacctggctgcagtacgtgattcttgatcccgagcttcgggttggaagtgggtgggagagttcgaggccttgcgcttaaggagccccttcgcctcgtgcttgagttgaggcctggcctgggcgctggggccgccgcgtgcgaatctggtggcaccttcgcgcctgtctcgctgctttcgataagtctctagccatttaaaatttttgatgacctgctgcgacgctttttttctggcaagatagtcttgtaaatgcgggccaagatctgcacactggtatttcggtttttggggccgcgggcggcgacggggcccgtgcgtcccagcgcacatgttcggcgaggcggggcctgcgagcgcggccaccgagaatcggacgggggtagtctcaagctggccggcctgctctggtgcctggcctcgcgccgccgtgtatcgccccgccctgggcggcaaggctggcccggtcggcaccagttgcgtgagcggaaagatggccgcttcccggccctgctgcagggagctcaaaatggaggacgcggcgctcgggagagcgggcgggtgagtcacccacacaaaggaaaagggcctttccgtcctcagccgtcgcttcatgtgactccactgagtaccgggcgccgtccaggcacctcgattagttctcgtgcttttggagtacgtcgtctttaggttggggggaggggttttatgcgatggagtttccccacactgagtgggtggagactgaagttaggccagcttggcacttgatgtaattctccttggaatttgccctttttgagtttggatcttggttcattctcaagcctcagacagtggttcaaagtttttttcttccatttcaggtgtcgtga

SEQ ID NO: 8 - DNA, 29 bp, synthetic construct
  misc_feature 1..29: note = Spacer + Kozak sequence
  source 1..29: mol_type = other DNA
ggcattccggtactgttggtaaagccacc

SEQ ID NO: 9 - DNA, 253 bp, synthetic construct
  misc_feature 1..253: note = Synthetic Construct
  source 1..253: mol_type = other DNA
ggaggaaaaactgtttcatacagaaggcgtggaggaaaaactgtttcatacagaaggcgtggaggaaaaactgtttcatacagaaggcgtggaggaaaaactgtttcatacagaaggcgtggaggaaaaactgtttcatacagaaggcgtggaggaaaaactgtttcatacagaaggcgtactagttagagggtatataatggaagctcgacttccagcccgggggcattccggtactgttggtaaagccacc

SEQ ID NO: 10 - DNA, 2936 bp, synthetic construct
  misc_feature 1..2936: note = pASP4.2
  source 1..2936: mol_type = other DNA
tcgagttaattaagctagcccggtactgttggaggaaaaactgtttcatacagaaggcgtggaggaaaaactgtttcatacagaaggcgtggaggaaaaactgtttcatacagaaggcgtggaggaaaaactgtttcatacagaaggcgtggaggaaaaactgtttcatacagaaggcgtggaggaaaaactgtttcatacagaaggcgtactagttagagggtatataatggaagctcgacttccagcccgggggcattccggtactgttggtaaagccaccatggtgagcaagggcgaggagctgttcaccggggtggtgcccatcctggtcgagctggacggcgacgtaaacggccacaagttcagcgtgtccggcgagggcgagggcgatgccacctacggcaagctgaccctgaagttcatctgcaccaccggcaagctgcccgtgccctggcccaccctcgtgaccaccctgacctacggcgtgcagtgcttcagccgctaccccgaccacatgaagcagcacgacttcttcaagtccgccatgcccgaaggctacgtccaggagcgcaccatcttcttcaaggacgacggcaactacaagacccgcgccgaggtgaagttcgagggcgacaccctggtgaaccgcatcgagctgaagggcatcgacttcaaggaggacggcaacatcctggggcacaagctggagtacaactacaacagccacaacgtctatatcatggccgacaagcagaagaacggcatcaaggtgaacttcaagatccgccacaacatcgaggacggcagcgtgcagctcgccgaccactaccagcagaacacccccatcggcgacggccccgtgctgctgcccgacaaccactacctgagcacccagtccgccctgagcaaagaccccaacgagaagcgcgatcacatggtcctgctggagttcgtgaccgccgccgggatcactctcggcatggacgagctgtacaagtaaatgcatcgtgaggctccggtgcccgtcagtgggcagagcgcacatcgcccacagtccccgagaagttggggggaggggtcggcaattgaaccggtgcctagagaaggtggcgcggggtaaactgggaaagtgatgtcgtgtactggctccgcctttttcccgagggtgggggagaaccgtatataagtgcagtagtcgccgtgaacgttctttttcgcaacgggtttgccgccagaacacaggtaagtgccgtgtgtggttcccgcgggcctggcctctttacgggttatggcccttgcgtgccttgaattacttccacctggctgcagtacgtgattcttgatcccgagcttcgggttggaagtgggtgggagagttcgaggccttgcgcttaaggagccccttcgcctcgtgcttgagttgaggcctggcctgggcgctggggccgccgcgtgcgaatctggtggcaccttcgcgcctgtctcgctgctttcgataagtctctagccatttaaaatttttgatgacctgctgcgacgctttttttctggcaagatagtcttgtaaatgcgggccaagatctgcacactggtatttcggtttttggggccgcgggcggcgacggggcccgtgcgtcccagcgcacatgttcggcgaggcggggcctgcgagcgcggccaccgagaatcggacgggggtagtctcaagctggccggcctgctctggtgcctggcctcgcgccgccgtgtatcgccccgccctgggcggcaaggctggcccggtcggcaccagttgcgtgagcggaaagatggccgcttcccggccctgctgcagggagctcaaaatggaggacgcggcgctcgggagagcgggcgggtgagtcacccacacaaaggaaaagggcctttccgtcctcagccgtcgcttcatgtgactccactgagtaccgggcgccgtccaggcacctcgattagttctcgtgcttttggagtacgtcgtctttaggttggggggaggggttttatgcgatggagtttccccacactgagtgggtggagactgaagttaggccagcttggcacttgatgtaattctccttggaatttgccctttttgagtttggatcttggttcattctcaagcctcagacagtggttcaaagtttttttcttccatttcaggtgtcgtgattctagagccaccatggtgagcaagggcgaggaggataacatggccatcatcaaggagttcatgcgcttcaaggtgcacatggagggctccgtgaacggccacgagttcgagatcgagggcgagggcgagggccgcccctacgagggcacccagaccgccaagctgaaggtgaccaagggtggccccctgcccttcgcctgggacatcctgtcccctcagttcatgtacggctccaaggcctacgtgaagcaccccgccgacatccccgactacttgaagctgtccttccccgagggcttcaagtgggagcgcgtgatgaacttcgaggacggcggcgtggtgaccgtgacccaggactcctccctgcaggacggcgagttcatctacaaggtgaagctgcgcggcaccaacttcccctccgacggccccgtaatgcagaagaagaccatgggctgggaggcctcctccgagcggatgtaccccgaggacggcgccctgaagggcgagatcaagcagaggctgaagctgaaggacggcggccactacgacgctgaggtcaagaccacctacaaggccaagaagcccgtgcagctgcccggcgcctacaacgtcaacatcaagttggacatcacctcccacaacgaggactacaccatcgtggaacagtacgaacgcgccgagggccgccactccaccggcggcatggacgagctgtacaagagggccaagaggcgtacgtaag

SEQ ID NO: 11 - DNA, 2936 bp, synthetic construct
  misc_feature 1..2936: note = pASP5
  source 1..2936: mol_type = other DNA
tcgagttaattaagctagcttacttgtacagctcgtccatgccgagagtgatcccggcggcggtcacgaactccagcaggaccatgtgatcgcgcttctcgttggggtctttgctcagggcggactgggtgctcaggtagtggttgtcgggcagcagcacggggccgtcgccgatgggggtgttctgctggtagtggtcggcgagctgcacgctgccgtcctcgatgttgtggcggatcttgaagttcaccttgatgccgttcttctgcttgtcggccatgatatagacgttgtggctgttgtagttgtactccagcttgtgccccaggatgttgccgtcctccttgaagtcgatgcccttcagctcgatgcggttcaccagggtgtcgccctcgaacttcacctcggcgcgggtcttgtagttgccgtcgtccttgaagaagatggtgcgctcctggacgtagccttcgggcatggcggacttgaagaagtcgtgctgcttcatgtggtcggggtagcggctgaagcactgcacgccgtaggtcagggtggtcacgagggtgggccagggcacgggcagcttgccggtggtgcagatgaacttcagggtcagcttgccgtaggtggcatcgccctcgccctcgccggacacgctgaacttgtggccgtttacgtcgccgtccagctcgaccaggatgggcaccaccccggtgaacagctcctcgcccttgctcaccatggtggctttaccaacagtaccggaatgcccccgggctggaagtcgagcttccattatataccctctaactagtacgccttctgtatgaaacagtttttcctccacgccttctgtatgaaacagtttttcctccacgccttctgtatgaaacagtttttcctccacgccttctgtatgaaacagtttttcctccacgccttctgtatgaaacagtttttcctccacgccttctgtatgaaacagtttttcctccaacagtaccggatgcatcgtgaggctccggtgcccgtcagtgggcagagcgcacatcgcccacagtccccgagaagttggggggaggggtcggcaattgaaccggtgcctagagaaggtggcgcggggtaaactgggaaagtgatgtcgtgtactggctccgcctttttcccgagggtgggggagaaccgtatataagtgcagtagtcgccgtgaacgttctttttcgcaacgggtttgccgccagaacacaggtaagtgccgtgtgtggttcccgcgggcctggcctctttacgggttatggcccttgcgtgccttgaattacttccacctggctgcagtacgtgattcttgatcccgagcttcgggttggaagtgggtgggagagttcgaggccttgcgcttaaggagccccttcgcctcgtgcttgagttgaggcctggcctgggcgctggggccgccgcgtgcgaatctggtggcaccttcgcgcctgtctcgctgctttcgataagtctctagccatttaaaatttttgatgacctgctgcgacgctttttttctggcaagatagtcttgtaaatgcgggccaagatctgcacactggtatttcggtttttggggccgcgggcggcgacggggcccgtgcgtcccagcgcacatgttcggcgaggcggggcctgcgagcgcggccaccgagaatcggacgggggtagtctcaagctggccggcctgctctggtgcctggcctcgcgccgccgtgtatcgccccgccctgggcggcaaggctggcccggtcggcaccagttgcgtgagcggaaagatggccgcttcccggccctgctgcagggagctcaaaatggaggacgcggcgctcgggagagcgggcgggtgagtcacccacacaaaggaaaagggcctttccgtcctcagccgtcgcttcatgtgactccactgagtaccgggcgccgtccaggcacctcgattagttctcgtgcttttggagtacgtcgtctttaggttggggggaggggttttatgcgatggagtttccccacactgagtgggtggagactgaagttaggccagcttggcacttgatgtaattctccttggaatttgccctttttgagtttggatcttggttcattctcaagcctcagacagtggttcaaagtttttttcttccatttcaggtgtcgtgattctagagccaccatggtgagcaagggcgaggaggataacatggccatcatcaaggagttcatgcgcttcaaggtgcacatggagggctccgtgaacggccacgagttcgagatcgagggcgagggcgagggccgcccctacgagggcacccagaccgccaagctgaaggtgaccaagggtggccccctgcccttcgcctgggacatcctgtcccctcagttcatgtacggctccaaggcctacgtgaagcaccccgccgacatccccgactacttgaagctgtccttccccgagggcttcaagtgggagcgcgtgatgaacttcgaggacggcggcgtggtgaccgtgacccaggactcctccctgcaggacggcgagttcatctacaaggtgaagctgcgcggcaccaacttcccctccgacggccccgtaatgcagaagaagaccatgggctgggaggcctcctccgagcggatgtaccccgaggacggcgccctgaagggcgagatcaagcagaggctgaagctgaaggacggcggccactacgacgctgaggtcaagaccacctacaaggccaagaagcccgtgcagctgcccggcgcctacaacgtcaacatcaagttggacatcacctcccacaacgaggactacaccatcgtggaacagtacgaacgcgccgagggccgccactccaccggcggcatggacgagctgtacaagagggccaagaggcgtacgtaag

SEQ ID NO: 12 - DNA, 3158 bp, synthetic construct
  misc_feature 1..3158: note = pASP7
  source 1..3158: mol_type = other DNA
tcgagtaccacatttgtagaggttttacttgctttaaaaaacctcccacacctccccctgaacctgaaacataaaatgaatgcaattgttgttgttaacttgtttattgcagcttataatggttacaaataaagcaatagcatcacaaatttcacaaataaagcatttttttcactgcattctagttgtggtttgtccaaactcatcaatgtatcttatcatgtctgttaattaagctagcttacttgtacagctcgtccatgccgagagtgatcccggcggcggtcacgaactccagcaggaccatgtgatcgcgcttctcgttggggtctttgctcagggcggactgggtgctcaggtagtggttgtcgggcagcagcacggggccgtcgccgatgggggtgttctgctggtagtggtcggcgagctgcacgctgccgtcctcgatgttgtggcggatcttgaagttcaccttgatgccgttcttctgcttgtcggccatgatatagacgttgtggctgttgtagttgtactccagcttgtgccccaggatgttgccgtcctccttgaagtcgatgcccttcagctcgatgcggttcaccagggtgtcgccctcgaacttcacctcggcgcgggtcttgtagttgccgtcgtccttgaagaagatggtgcgctcctggacgtagccttcgggcatggcggacttgaagaagtcgtgctgcttcatgtggtcggggtagcggctgaagcactgcacgccgtaggtcagggtggtcacgagggtgggccagggcacgggcagcttgccggtggtgcagatgaacttcagggtcagcttgccgtaggtggcatcgccctcgccctcgccggacacgctgaacttgtggccgtttacgtcgccgtccagctcgaccaggatgggcaccaccccggtgaacagctcctcgcccttgctcaccatggtggctttaccaacagtaccggaatgcccccgggctggaagtcgagcttccattatataccctctaactagtacgccttctgtatgaaacagtttttcctccacgccttctgtatgaaacagtttttcctccacgccttctgtatgaaacagtttttcctccacgccttctgtatgaaacagtttttcctccacgccttctgtatgaaacagtttttcctccacgccttctgtatgaaacagtttttcctccaacagtaccggatgcatcgtgaggctccggtgcccgtcagtgggcagagcgcacatcgcccacagtccccgagaagttggggggaggggtcggcaattgaaccggtgcctagagaaggtggcgcggggtaaactgggaaagtgatgtcgtgtactggctccgcctttttcccgagggtgggggagaaccgtatataagtgcagtagtcgccgtgaacgttctttttcgcaacgggtttgccgccagaacacaggtaagtgccgtgtgtggttcccgcgggcctggcctctttacgggttatggcccttgcgtgccttgaattacttccacctggctgcagtacgtgattcttgatcccgagcttcgggttggaagtgggtgggagagttcgaggccttgcgcttaaggagccccttcgcctcgtgcttgagttgaggcctggcctgggcgctggggccgccgcgtgcgaatctggtggcaccttcgcgcctgtctcgctgctttcgataagtctctagccatttaaaatttttgatgacctgctgcgacgctttttttctggcaagatagtcttgtaaatgcgggccaagatctgcacactggtatttcggtttttggggccgcgggcggcgacggggcccgtgcgtcccagcgcacatgttcggcgaggcggggcctgcgagcgcggccaccgagaatcggacgggggtagtctcaagctggccggcctgctctggtgcctggcctcgcgccgccgtgtatcgccccgccctgggcggcaaggctggcccggtcggcaccagttgcgtgagcggaaagatggccgcttcccggccctgctgcagggagctcaaaatggaggacgcggcgctcgggagagcgggcgggtgagtcacccacacaaaggaaaagggcctttccgtcctcagccgtcgcttcatgtgactccactgagtaccgggcgccgtccaggcacctcgattagttctcgtgcttttggagtacgtcgtctttaggttggggggaggggttttatgcgatggagtttccccacactgagtgggtggagactgaagttaggccagcttggcacttgatgtaattctccttggaatttgccctttttgagtttggatcttggttcattctcaagcctcagacagtggttcaaagtttttttcttccatttcaggtgtcgtgattctagagccaccatggtgagcaagggcgaggaggataacatggccatcatcaaggagttcatgcgcttcaaggtgcacatggagggctccgtgaacggccacgagttcgagatcgagggcgagggcgagggccgcccctacgagggcacccagaccgccaagctgaaggtgaccaagggtggccccctgcccttcgcctgggacatcctgtcccctcagttcatgtacggctccaaggcctacgtgaagcaccccgccgacatccccgactacttgaagctgtccttccccgagggcttcaagtgggagcgcgtgatgaacttcgaggacggcggcgtggtgaccgtgacccaggactcctccctgcaggacggcgagttcatctacaaggtgaagctgcgcggcaccaacttcccctccgacggccccgtaatgcagaagaagaccatgggctgggaggcctcctccgagcggatgtaccccgaggacggcgccctgaagggcgagatcaagcagaggctgaagctgaaggacggcggccactacgacgctgaggtcaagaccacctacaaggccaagaagcccgtgcagctgcccggcgcctacaacgtcaacatcaagttggacatcacctcccacaacgaggactacaccatcgtggaacagtacgaacgcgccgagggccgccactccaccggcggcatggacgagctgtacaagagggccaagaggcgtacgtaag

SEQ ID NO: 13 - DNA, 3413 bp, synthetic construct
  misc_feature 1..3413: note = pASP8
  source 1..3413: mol_type = other DNA
tcgagttaattaagctagcaaggctttctgtttcctgcattcttacttcttactacgtgatacatctagtcaccagggaagaagcgaatgacacacttccaaaaaccaattcgtagctttctaaataaaaccctttctagctggagagagatccatgagcatagagatcttaaaattcatgttcagcaataaatcctggggccccagacagtgtcaggtgcatagggggtgttcagtaaatatcagttaaatgttgcataaatccgataaacgggattcctggaaaatactacactctccttctccaaattatcttcatctcaaagacaggaacctctaacttttaattctttacttagattatgctgtctcctaaactgtttatgttttctgaaatttaaggcaggatgtctcagagtctgggaaaatcccactttcctcctgctacaccttacagttgtgagaaagcacatttcagacaacagggaaaacccatacttcaccacaacaacacactatacattgtctggtccactggagcataaattaaagagaaacaatgtagtcaagcaagtaggcggcaagaggaagggggcggagacatcatcagggagtataaactctgagatgcctcagagcctcacagactcaacaagagctccagcaaagactttcactgtagcttgacttgacctgagattaactagggaatcttgagaataaagcccgggggcattccggtactgttggtaaagccaccatggtgagcaagggcgaggagctgttcaccggggtggtgcccatcctggtcgagctggacggcgacgtaaacggccacaagttcagcgtgtccggcgagggcgagggcgatgccacctacggcaagctgaccctgaagttcatctgcaccaccggcaagctgcccgtgccctggcccaccctcgtgaccaccctgacctacggcgtgcagtgcttcagccgctaccccgaccacatgaagcagcacgacttcttcaagtccgccatgcccgaaggctacgtccaggagcgcaccatcttcttcaaggacgacggcaactacaagacccgcgccgaggtgaagttcgagggcgacaccctggtgaaccgcatcgagctgaagggcatcgacttcaaggaggacggcaacatcctggggcacaagctggagtacaactacaacagccacaacgtctatatcatggccgacaagcagaagaacggcatcaaggtgaacttcaagatccgccacaacatcgaggacggcagcgtgcagctcgccgaccactaccagcagaacacccccatcggcgacggccccgtgctgctgcccgacaaccactacctgagcacccagtccgccctgagcaaagaccccaacgagaagcgcgatcacatggtcctgctggagttcgtgaccgccgccgggatcactctcggcatggacgagctgtacaagtaaatgcatcgtgaggctccggtgcccgtcagtgggcagagcgcacatcgcccacagtccccgagaagttggggggaggggtcggcaattgaaccggtgcctagagaaggtggcgcggggtaaactgggaaagtgatgtcgtgtactggctccgcctttttcccgagggtgggggagaaccgtatataagtgcagtagtcgccgtgaacgttctttttcgcaacgggtttgccgccagaacacaggtaagtgccgtgtgtggttcccgcgggcctggcctctttacgggttatggcccttgcgtgccttgaattacttccacctggctgcagtacgtgattcttgatcccgagcttcgggttggaagtgggtgggagagttcgaggccttgcgcttaaggagccccttcgcctcgtgcttgagttgaggcctggcctgggcgctggggccgccgcgtgcgaatctggtggcaccttcgcgcctgtctcgctgctttcgataagtctctagccatttaaaatttttgatgacctgctgcgacgctttttttctggcaagatagtcttgtaaatgcgggccaagatctgcacactggtatttcggtttttggggccgcgggcggcgacggggcccgtgcgtcccagcgcacatgttcggcgaggcggggcctgcgagcgcggccaccgagaatcggacgggggtagtctcaagctggccggcctgctctggtgcctggcctcgcgccgccgtgtatcgccccgccctgggcggcaaggctggcccggtcggcaccagttgcgtgagcggaaagatggccgcttcccggccctgctgcagggagctcaaaatggaggacgcggcgctcgggagagcgggcgggtgagtcacccacacaaaggaaaagggcctttccgtcctcagccgtcgcttcatgtgactccactgagtaccgggcgccgtccaggcacctcgattagttctcgtgcttttggagtacgtcgtctttaggttggggggaggggttttatgcgatggagtttccccacactgagtgggtggagactgaagttaggccagcttggcacttgatgtaattctccttggaatttgccctttttgagtttggatcttggttcattctcaagcctcagacagtggttcaaagtttttttcttccatttcaggtgtcgtgattctagagccaccatggtgagcaagggcgaggaggataacatggccatcatcaaggagttcatgcgcttcaaggtgcacatggagggctccgtgaacggccacgagttcgagatcgagggcgagggcgagggccgcccctacgagggcacccagaccgccaagctgaaggtgaccaagggtggccccctgcccttcgcctgggacatcctgtcccctcagttcatgtacggctccaaggcctacgtgaagcaccccgccgacatccccgactacttgaagctgtccttccccgagggcttcaagtgggagcgcgtgatgaacttcgaggacggcggcgtggtgaccgtgacccaggactcctccctgcaggacggcgagttcatctacaaggtgaagctgcgcggcaccaacttcccctccgacggccccgtaatgcagaagaagaccatgggctgggaggcctcctccgagcggatgtaccccgaggacggcgccctgaagggcgagatcaagcagaggctgaagctgaaggacggcggccactacgacgctgaggtcaagaccacctacaaggccaagaagcccgtgcagctgcccggcgcctacaacgtcaacatcaagttggacatcacctcccacaacgaggactacaccatcgtggaacagtacgaacgcgccgagggccgccactccaccggcggcatggacgagctgtacaagagggccaagaggcgtacgtaag

SEQ ID NO: 14 - DNA, 3031 bp, synthetic construct
  misc_feature 1..3031: note = pASP9
  source 1..3031: mol_type = other DNA
tcgagttaattaagctagcaatgctttgtcctggagagctatcttaagggacaaaatcgttttcccagcgtcatctgtgacacatcctgacagtagagagctgcttccaagaagcaatttgaagtgccattatcaggcagggacgggggctctaggggatttcggggtcagcagatatgaaatgaatgatttcatagggctgtcacagagctgtggtgggaatttcccatgagaccccgcccctggctgagtcaccgcactcctgtgtttgacctgaagtcctctcgtgctgcagaagcctgaagaccaaggagtggaaagttctccggcagccctgagatctcccgggggcattccggtactgttggtaaagccaccatggtgagcaagggcgaggagctgttcaccggggtggtgcccatcctggtcgagctggacggcgacgtaaacggccacaagttcagcgtgtccggcgagggcgagggcgatgccacctacggcaagctgaccctgaagttcatctgcaccaccggcaagctgcccgtgccctggcccaccctcgtgaccaccctgacctacggcgtgcagtgcttcagccgctaccccgaccacatgaagcagcacgacttcttcaagtccgccatgcccgaaggctacgtccaggagcgcaccatcttcttcaaggacgacggcaactacaagacccgcgccgaggtgaagttcgagggcgacaccctggtgaaccgcatcgagctgaagggcatcgacttcaaggaggacggcaacatcctggggcacaagctggagtacaactacaacagccacaacgtctatatcatggccgacaagcagaagaacggcatcaaggtgaacttcaagatccgccacaacatcgaggacggcagcgtgcagctcgccgaccactaccagcagaacacccccatcggcgacggccccgtgctgctgcccgacaaccactacctgagcacccagtccgccctgagcaaagaccccaacgagaagcgcgatcacatggtcctgctggagttcgtgaccgccgccgggatcactctcggcatggacgagctgtacaagtaaatgcatcgtgaggctccggtgcccgtcagtgggcagagcgcacatcgcccacagtccccgagaagttggggggaggggtcggcaattgaaccggtgcctagagaaggtggcgcggggtaaactgggaaagtgatgtcgtgtactggctccgcctttttcccgagggtgggggagaaccgtatataagtgcagtagtcgccgtgaacgttctttttcgcaacgggtttgccgccagaacacaggtaagtgccgtgtgtggttcccgcgggcctggcctctttacgggttatggcccttgcgtgccttgaattacttccacctggctgcagtacgtgattcttgatcccgagcttcgggttggaagtgggtgggagagttcgaggccttgcgcttaaggagccccttcgcctcgtgcttgagttgaggcctggcctgggcgctggggccgccgcgtgcgaatctggtggcaccttcgcgcctgtctcgctgctttcgataagtctctagccatttaaaatttttgatgacctgctgcgacgctttttttctggcaagatagtcttgtaaatgcgggccaagatctgcacactggtatttcggtttttggggccgcgggcggcgacggggcccgtgcgtcccagcgcacatgttcggcgaggcggggcctgcgagcgcggccaccgagaatcggacgggggtagtctcaagctggccggcctgctctggtgcctggcctcgcgccgccgtgtatcgccccgccctgggcggcaaggctggcccggtcggcaccagttgcgtgagcggaaagatggccgcttcccggccctgctgcagggagctcaaaatggaggacgcggcgctcgggagagcgggcgggtgagtcacccacacaaaggaaaagggcctttccgtcctcagccgtcgcttcatgtgactccactgagtaccgggcgccgtccaggcacctcgattagttctcgtgcttttggagtacgtcgtctttaggttggggggaggggttttatgcgatggagtttccccacactgagtgggtggagactgaagttaggccagcttggcacttgatgtaattctccttggaatttgccctttttgagtttggatcttggttcattctcaagcctcagacagtggttcaaagtttttttcttccatttcaggtgtcgtgattctagagccaccatggtgagcaagggcgaggaggataacatggccatcatcaaggagttcatgcgcttcaaggtgcacatggagggctccgtgaacggccacgagttcgagatcgagggcgagggcgagggccgcccctacgagggcacccagaccgccaagctgaaggtgaccaagggtggccccctgcccttcgcctgggacatcctgtcccctcagttcatgtacggctccaaggcctacgtgaagcaccccgccgacatccccgactacttgaagctgtccttccccgagggcttcaagtgggagcgcgtgatgaacttcgaggacggcggcgtggtgaccgtgacccaggactcctccctgcaggacggcgagttcatctacaaggtgaagctgcgcggcaccaacttcccctccgacggccccgtaatgcagaagaagaccatgggctgggaggcctcctccgagcggatgtaccccgaggacggcgccctgaagggcgagatcaagcagaggctgaagctgaaggacggcggccactacgacgctgaggtcaagaccacctacaaggccaagaagcccgtgcagctgcccggcgcctacaacgtcaacatcaagttggacatcacctcccacaacgaggactacaccatcgtggaacagtacgaacgcgccgagggccgccactccaccggcggcatggacgagctgtacaagagggccaagaggcgtacgtaag

SEQ ID NO: 15 - DNA, 3815 bp, synthetic construct
  misc_feature 1..3815: note = pASP18
  source 1..3815: mol_type = other DNA
tcgagttaattaagctagcccggtactgttggaggaaaaactgtttcatacagaaggcgtggaggaaaaactgtttcatacagaaggcgtggaggaaaaactgtttcatacagaaggcgtggaggaaaaactgtttcatacagaaggcgtggaggaaaaactgtttcatacagaaggcgtggaggaaaaactgtttcatacagaaggcgtactagttagagggtatataatggaagctcgacttccagcccgggggcattccggtactgttggtaaagccaccatgtgccaccagcagctggtcatcagctggttcagcctggtgttcctggccagccctctggtggccatctgggagctgaagaaagacgtgtacgtggtggaactggactggtatcccgacgcccctggcgagatggtggtgctgacctgcgacacccctgaagaggacggcatcacctggaccctggaccagtctagcgaggtgctgggcagcggcaagaccctgaccatccaggtcaaagagttcggcgacgccggccagtacacctgtcacaagggcggagaggtgctgagccacagcctgctgctgctccacaagaaagaggatggcatttggagcaccgacatcctgaaggaccagaaagagcccaagaacaagaccttcctgagatgcgaggccaagaactacagcggccggttcacctgttggtggctgaccaccatcagcaccgacctgaccttcagcgtgaagtccagcagaggcagcagcgaccctcagggcgtgacatgtggcgccgctacactgtctgccgagagagtgcggggcgacaacaaagagtacgagtacagcgtcgagtgccaggaagatagcgcctgccctgccgccgaggaaagcctgcctatcgaagtgatggtggacgccgtgcacaagctgaagtacgagaactacacctccagctttttcatccgggacatcatcaagcccgaccctcccaagaacctgcagctgaagcctctgaagaacagcagacaggtggaagtgtcctgggagtaccccgacacctggtccacccctcacagctacttcagcctgacattctgtgtgcaagtccagggcaagtccaagcgcgagaaaaaggaccgggtgttcaccgacaagaccagcgccaccgtgatctgccggaagaacgcctctatcagcgtgcgggcccaggaccggtactacagcagctcttggagcgagtgggccagcgtgccatgttctggtggcggaggcggcggaagcagaaatctgccagtggccacccctgaccccggcatgtttccttgtctgcaccacagccagaacctgctgcgggccgtgtccaacatgctgcagaaggcccggcagaccctggaattctacccctgcaccagcgaggaaatcgaccacgaggacatcaccaaggataagaccagcaccgtggaagcctgtctgcccctggaactgaccaagaacgagagctgcctgaacagccgggaaaccagcttcatcaccaacggcagctgtctggccagcagaaagacctccttcatgatggccctgtgcctgagcagcatctacgaggacctgaagatgtaccaggtcgagttcaagaccatgaacgccaagctgctgatggaccccaagcggcagatctttctggaccagaatatgctggccgtgatcgacgagctgatgcaggccctgaacttcaacagcgagacagtgccccagaagtcctccctggaagaacccgacttctacaagaccaagatcaagctgtgcatcctgctgcacgccttccggatcagagccgtgaccatcgacagagtgatgagctacctgaacgcctcctaaatgcatcgtgaggctccggtgcccgtcagtgggcagagcgcacatcgcccacagtccccgagaagttggggggaggggtcggcaattgaaccggtgcctagagaaggtggcgcggggtaaactgggaaagtgatgtcgtgtactggctccgcctttttcccgagggtgggggagaaccgtatataagtgcagtagtcgccgtgaacgttctttttcgcaacgggtttgccgccagaacacaggtaagtgccgtgtgtggttcccgcgggcctggcctctttacgggttatggcccttgcgtgccttgaattacttccacctggctgcagtacgtgattcttgatcccgagcttcgggttggaagtgggtgggagagttcgaggccttgcgcttaaggagccccttcgcctcgtgcttgagttgaggcctggcctgggcgctggggccgccgcgtgcgaatctggtggcaccttcgcgcctgtctcgctgctttcgataagtctctagccatttaaaatttttgatgacctgctgcgacgctttttttctggcaagatagtcttgtaaatgcgggccaagatctgcacactggtatttcggtttttggggccgcgggcggcgacggggcccgtgcgtcccagcgcacatgttcggcgaggcggggcctgcgagcgcggccaccgagaatcggacgggggtagtctcaagctggccggcctgctctggtgcctggcctcgcgccgccgtgtatcgccccgccctgggcggcaaggctggcccggtcggcaccagttgcgtgagcggaaagatggccgcttcccggccctgctgcagggagctcaaaatggaggacgcggcgctcgggagagcgggcgggtgagtcacccacacaaaggaaaagggcctttccgtcctcagccgtcgcttcatgtgactccactgagtaccgggcgccgtccaggcacctcgattagttctcgtgcttttggagtacgtcgtctttaggttggggggaggggttttatgcgatggagtttccccacactgagtgggtggagactgaagttaggccagcttggcacttgatgtaattctccttggaatttgccctttttgagtttggatcttggttcattctcaagcctcagacagtggttcaaagtttttttcttccatttcaggtgtcgtgattctagagccaccatggtgagcaagggcgaggaggataacatggccatcatcaaggagttcatgcgcttcaaggtgcacatggagggctccgtgaacggccacgagttcgagatcgagggcgagggcgagggccgcccctacgagggcacccagaccgccaagctgaaggtgaccaagggtggccccctgcccttcgcctgggacatcctgtcccctcagttcatgtacggctccaaggcctacgtgaagcaccccgccgacatccccgactacttgaagctgtccttccccgagggcttcaagtgggagcgcgtgatgaacttcgaggacggcggcgtggtgaccgtgacccaggactcctccctgcaggacggcgagttcatctacaaggtgaagctgcgcggcaccaacttcccctccgacggccccgtaatgcagaagaagaccatgggctgggaggcctcctccgagcggatgtaccccgaggacggcgccctgaagggcgagatcaagcagaggctgaagctgaaggacggcggccactacgacgctgaggtcaagaccacctacaaggccaagaagcccgtgcagctgcccggcgcctacaacgtcaacatcaagttggacatcacctcccacaacgaggactacaccatcgtggaacagtacgaacgcgccgagggccgccactccaccggcggcatggacgagctgtacaagagggccaagaggcgtacgtaag

SEQ ID NO: 16 - DNA, 3680 bp, synthetic construct
  misc_feature 1..3680: note = pASP26
  source 1..3680: mol_type = other DNA
tcgagttaattaagctagcccggtactgttggaggaaaaactgtttcatacagaaggcgtggaggaaaaactgtttcatacagaaggcgtggaggaaaaactgtttcatacagaaggcgtggaggaaaaactgtttcatacagaaggcgtggaggaaaaactgtttcatacagaaggcgtggaggaaaaactgtttcatacagaaggcgtactagttagagggtatataatggaagctcgacttccagcccgggggcattccggtactgttggtaaagccaccatggtgagcaagggcgaggagctgttcaccggggtggtgcccatcctggtcgagctggacggcgacgtaaacggccacaagttcagcgtgtccggcgagggcgagggcgatgccacctacggcaagctgaccctgaagttcatctgcaccaccggcaagctgcccgtgccctggcccaccctcgtgaccaccctgacctacggcgtgcagtgcttcagccgctaccccgaccacatgaagcagcacgacttcttcaagtccgccatgcccgaaggctacgtccaggagcgcaccatcttcttcaaggacgacggcaactacaagacccgcgccgaggtgaagttcgagggcgacaccctggtgaaccgcatcgagctgaagggcatcgacttcaaggaggacggcaacatcctggggcacaagctggagtacaactacaacagccacaacgtctatatcatggccgacaagcagaagaacggcatcaaggtgaacttcaagatccgccacaacatcgaggacggcagcgtgcagctcgccgaccactaccagcagaacacccccatcggcgacggccccgtgctgctgcccgacaaccactacctgagcacccagtccgccctgagcaaagaccccaacgagaagcgcgatcacatggtcctgctggagttcgtgaccgccgccgggatcactctcggcatggacgagctgtacaagtaaatgcatcgtgaggctccggtgcccgtcagtgggcagagcgcacatcgcccacagtccccgagaagttggggggaggggtcggcaattgaaccggtgcctagagaaggtggcgcggggtaaactgggaaagtgatgtcgtgtactggctccgcctttttcccgagggtgggggagaaccgtatataagtgcagtagtcgccgtgaacgttctttttcgcaacgggtttgccgccagaacacaggtaagtgccgtgtgtggttcccgcgggcctggcctctttacgggttatggcccttgcgtgccttgaattacttccacctggctgcagtacgtgattcttgatcccgagcttcgggttggaagtgggtgggagagttcgaggccttgcgcttaaggagccccttcgcctcgtgcttgagttgaggcctggcctgggcgctggggccgccgcgtgcgaatctggtggcaccttcgcgcctgtctcgctgctttcgataagtctctagccatttaaaatttttgatgacctgctgcgacgctttttttctggcaagatagtcttgtaaatgcgggccaagatctgcacactggtatttcggtttttggggccgcgggcggcgacggggcccgtgcgtcccagcgcacatgttcggcgaggcggggcctgcgagcgcggccaccgagaatcggacgggggtagtctcaagctggccggcctgctctggtgcctggcctcgcgccgccgtgtatcgccccgccctgggcggcaaggctggcccggtcggcaccagttgcgtgagcggaaagatggccgcttcccggccctgctgcagggagctcaaaatggaggacgcggcgctcgggagagcgggcgggtgagtcacccacacaaaggaaaagggcctttccgtcctcagccgtcgcttcatgtgactccactgagtaccgggcgccgtccaggcacctcgattagttctcgtgcttttggagtacgtcgtctttaggttggggggaggggttttatgcgatggagtttccccacactgagtgggtggagactgaagttaggccagcttggcacttgatgtaattctccttggaatttgccctttttgagtttggatcttggttcattctcaagcctcagacagtggttcaaagtttttttcttccatttcaggtgtcgtgattctagagccaccatggccttaccagtgaccgccttgctcctgccgctggccttgctgctccacgccgccaggccggacattcaaatgacacagagtccctcatccctcagtgccagcgtgggcgatcgggtgactataacctgcagagcttctcaggacgtgaataccgctgtggcgtggtaccagcagaagccaggcaaagcgcctaagcttctcatttatagtgccagcttcctgtactcaggtgttccgtctcgcttttctggaagtagaagtgggaccgatttcacattgacgatcagcagcttgcagcccgaagatttcgccacctactactgtcagcagcactacactaccccaccgacatttggtcaaggcacaaaagtagagattaaacgcactggttccaccagcgggagcgggaaacccggctctggggaggggagcgaggtccagctggtggaatccgggggtggtcttgtgcagccaggaggatccttgaggttgtcctgcgccgcaagcggctttaacatcaaagatacatacatccattgggtccgacaggcccctggaaagggcctggagtgggtcgcccggatctacccaactaacgggtacactcgctacgctgatagcgtcaagggtcggtttactatttctgccgacacctcaaaaaacacagcctacctccagatgaactctctcagagctgaggatacagccgtgtactattgcagccggtggggaggcgacgggttctacgctatggatgtgtgggggcagggcacactggtcaccgtgagctcatccggaaccacgacgccagcgccgcgaccaccaacaccggcgcccaccatcgcgtcgcagcccctgtccctgcgcccagaggcgtgccggccagcggcggggggcgcagtgcacacgagggggctggacttcgcctgtgatatctacatctgggcgcccttggccgggacttgtggggtccttctcctgtcactggttatcaccctttactgcaaacggggcagaaagaaactcctgtatatattcaaacaaccatttatgagaccagtacaaactactcaagaggaagatggctgtagctgccgatttccagaagaagaagaaggaggatgtgaactgagagtgaagttcagcaggagcgcagacgcccccgcgtacaagcagggccagaaccagctctataacgagctcaatctaggacgaagagaggagtacgatgttttggacaagagacgtggccgggaccctgagatggggggaaagccgagaaggaagaaccctcaggaaggcctgtacaatgaactgcagaaagataagatggcggaggcctacagtgagattgggatgaaaggcgagcgccggaggggcaaggggcacgatggcctttaccagggtctcagtacagccaccaaggacacctacgacgcccttcacatgcaggccctgccccctcgctaag

SEQ ID NO: 17 - DNA, 3689 bp, synthetic construct
  misc_feature 1..3689: note = pASP28
  source 1..3689: mol_type = other DNA
tcgagttaattaagctagcttacttgtacagctcgtccatgccgagagtgatcccggcggcggtcacgaactccagcaggaccatgtgatcgcgcttctcgttggggtctttgctcagggcggactgggtgctcaggtagtggttgtcgggcagcagcacggggccgtcgccgatgggggtgttctgctggtagtggtcggcgagctgcacgctgccgtcctcgatgttgtggcggatcttgaagttcaccttgatgccgttcttctgcttgtcggccatgatatagacgttgtggctgttgtagttgtactccagcttgtgccccaggatgttgccgtcctccttgaagtcgatgcccttcagctcgatgcggttcaccagggtgtcgccctcgaacttcacctcggcgcgggtcttgtagttgccgtcgtccttgaagaagatggtgcgctcctggacgtagccttcgggcatggcggacttgaagaagtcgtgctgcttcatgtggtcggggtagcggctgaagcactgcacgccgtaggtcagggtggtcacgagggtgggccagggcacgggcagcttgccggtggtgcagatgaacttcagggtcagcttgccgtaggtggcatcgccctcgccctcgccggacacgctgaacttgtggccgtttacgtcgccgtccagctcgaccaggatgggcaccaccccggtgaacagctcctcgcccttgctcaccatggtggctttaccaacagtaccggaatgcccccgggctggaagtcgagcttccattatataccctctaactagtacgccttctgtatgaaacagtttttcctccacgccttctgtatgaaacagtttttcctccacgccttctgtatgaaacagtttttcctccacgccttctgtatgaaacagtttttcctccacgccttctgtatgaaacagtttttcctccacgccttctgtatgaaacagtttttcctccaacagtaccggatgcatcgtgaggctccggtgcccgtcagtgggcagagcgcacatcgcccacagtccccgagaagttggggggaggggtcggcaattgaaccggtgcctagagaaggtggcgcggggtaaactgggaaagtgatgtcgtgtactggctccgcctttttcccgagggtgggggagaaccgtatataagtgcagtagtcgccgtgaacgttctttttcgcaacgggtttgccgccagaacacaggtaagtgccgtgtgtggttcccgcgggcctggcctctttacgggttatggcccttgcgtgccttgaattacttccacctggctgcagtacgtgattcttgatcccgagcttcgggttggaagtgggtgggagagttcgaggccttgcgcttaaggagccccttcgcctcgtgcttgagttgaggcctggcctgggcgctggggccgccgcgtgcgaatctggtggcaccttcgcgcctgtctcgctgctttcgataagtctctagccatttaaaatttttgatgacctgctgcgacgctttttttctggcaagatagtcttgtaaatgcgggccaagatctgcacactggtatttcggtttttggggccgcgggcggcgacggggcccgtgcgtcccagcgcacatgttcggcgaggcggggcctgcgagcgcggccaccgagaatcggacgggggtagtctcaagctggccggcctgctctggtgcctggcctcgcgccgccgtgtatcgccccgccctgggcggcaaggctggcccggtcggcaccagttgcgtgagcggaaagatggccgcttcccggccctgctgcagggagctcaaaatggaggacgcggcgctcgggagagcgggcgggtgagtcacccacacaaaggaaaagggcctttccgtcctcagccgtcgcttcatgtgactccactgagtaccgggcgccgtccaggcacctcgattagttctcgtgcttttggagtacgtcgtctttaggttggggggaggggttttatgcgatggagtttccccacactgagtgggtggagactgaagttaggccagcttggcacttgatgtaattctccttggaatttgccctttttgagtttggatcttggttcattctcaagcctcagacagtggttcaaagtttttttcttccatttcaggtgtcgtgattctagaatggccttaccagtgaccgccttgctcctgccgctggccttgctgctccacgccgccaggccgggatccgacatcgttctgagtcagagccccgccatactgagcgcctcccccggggagaaggtgaccatgacctgtagagccagctccagcctttcatttatgcactggtaccagcagaaacccggtagtagtccaaagccgtggatttacgctacatccaacctggcaagcggagtaccagcccgcttctccggcagcggatcaggaacctcctactccctgacaatcagccgcgtcgaagccgaggatgcagccacatacttttgccaccagtggtcctctaatcccctgacatttggcgcaggcaccaagctcgaactgaagcggggatctaccagcggcagtggaaaacctggtagcggagaggggtctaccaaggggcaagtgcaactcagacagcctggcgcagaactcgtgaagcccggcgcatccgtcaagatgtcttgtaaagccagtggctacaccttcactagctataatatgcactgggttaaacagactcccggtcagggcctcgagtggattggcgcaatctacccgggtaatggtgatacttcttacaatcagaagtttaaggggaaagctaccctgaccgccgacaagtcttcatcaaccgcctacatgcagctgagctctctgacgtctgaggattccgccgtgtattactgcgcccggagccactacgggagtaattatgtcgattattttgactactggggtcagggaacaaccctgactgtctccagctccggaaccacgacgccagcgccgcgaccaccaacaccggcgcccaccatcgcgtcgcagcccctgtccctgcgcccagaggcgtgccggccagcggcggggggcgcagtgcacacgagggggctggacttcgcctgtgatatctacatctgggcgcccttggccgggacttgtggggtccttctcctgtcactggttatcaccctttactgcaaacggggcagaaagaaactcctgtatatattcaaacaaccatttatgagaccagtacaaactactcaagaggaagatggctgtagctgccgatttccagaagaagaagaaggaggatgtgaactgagagtgaagttcagcaggagcgcagacgcccccgcgtacaagcagggccagaaccagctctataacgagctcaatctaggacgaagagaggagtacgatgttttggacaagagacgtggccgggaccctgagatggggggaaagccgagaaggaagaaccctcaggaaggcctgtacaatgaactgcagaaagataagatggcggaggcctacagtgagattgggatgaaaggcgagcgccggaggggcaaggggcacgatggcctttaccagggtctcagtacagccaccaaggacacctacgacgcccttcacatgcaggccctgccccctcgctaag

SEQ ID NO: 18 - DNA, 3680 bp, synthetic construct
  misc_feature 1..3680: note = pASP30
  source 1..3680: mol_type = other DNA
tcgagttaattaagctagcttacttgtacagctcgtccatgccgagagtgatcccggcggcggtcacgaactccagcaggaccatgtgatcgcgcttctcgttggggtctttgctcagggcggactgggtgctcaggtagtggttgtcgggcagcagcacggggccgtcgccgatgggggtgttctgctggtagtggtcggcgagctgcacgctgccgtcctcgatgttgtggcggatcttgaagttcaccttgatgccgttcttctgcttgtcggccatgatatagacgttgtggctgttgtagttgtactccagcttgtgccccaggatgttgccgtcctccttgaagtcgatgcccttcagctcgatgcggttcaccagggtgtcgccctcgaacttcacctcggcgcgggtcttgtagttgccgtcgtccttgaagaagatggtgcgctcctggacgtagccttcgggcatggcggacttgaagaagtcgtgctgcttcatgtggtcggggtagcggctgaagcactgcacgccgtaggtcagggtggtcacgagggtgggccagggcacgggcagcttgccggtggtgcagatgaacttcagggtcagcttgccgtaggtggcatcgccctcgccctcgccggacacgctgaacttgtggccgtttacgtcgccgtccagctcgaccaggatgggcaccaccccggtgaacagctcctcgcccttgctcaccatggtggctttaccaacagtaccggaatgcccccgggctggaagtcgagcttccattatataccctctaactagtacgccttctgtatgaaacagtttttcctccacgccttctgtatgaaacagtttttcctccacgccttctgtatgaaacagtttttcctccacgccttctgtatgaaacagtttttcctccacgccttctgtatgaaacagtttttcctccacgccttctgtatgaaacagtttttcctccaacagtaccggatgcatcgtgaggctccggtgcccgtcagtgggcagagcgcacatcgcccacagtccccgagaagttggggggaggggtcggcaattgaaccggtgcctagagaaggtggcgcggggtaaactgggaaagtgatgtcgtgtactggctccgcctttttcccgagggtgggggagaaccgtatataagtgcagtagtcgccgtgaacgttctttttcgcaacgggtttgccgccagaacacaggtaagtgccgtgtgtggttcccgcgggcctggcctctttacgggttatggcccttgcgtgccttgaattacttccacctggctgcagtacgtgattcttgatcccgagcttcgggttggaagtgggtgggagagttcgaggccttgcgcttaaggagccccttcgcctcgtgcttgagttgaggcctggcctgggcgctggggccgccgcgtgcgaatctggtggcaccttcgcgcctgtctcgctgctttcgataagtctctagccatttaaaatttttgatgacctgctgcgacgctttttttctggcaagatagtcttgtaaatgcgggccaagatctgcacactggtatttcggtttttggggccgcgggcggcgacggggcccgtgcgtcccagcgcacatgttcggcgaggcggggcctgcgagcgcggccaccgagaatcggacgggggtagtctcaagctggccggcctgctctggtgcctggcctcgcgccgccgtgtatcgccccgccctgggcggcaaggctggcccggtcggcaccagttgcgtgagcggaaagatggccgcttcccggccctgctgcagggagctcaaaatggaggacgcggcgctcgggagagcgggcgggtgagtcacccacacaaaggaaaagggcctttccgtcctcagccgtcgcttcatgtgactccactgagtaccgggcgccgtccaggcacctcgattagttctcgtgcttttggagtacgtcgtctttaggttggggggaggggttttatgcgatggagtttccccacactgagtgggtggagactgaagttaggccagcttggcacttgatgtaattctccttggaatttgccctttttgagtttggatcttggttcattctcaagcctcagacagtggttcaaagtttttttcttccatttcaggtgtcgtgattctagagccaccatggccttaccagtgaccgccttgctcctgccgctggccttgctgctccacgccgccaggccggacattcaaatgacacagagtccctcatccctcagtgccagcgtgggcgatcgggtgactataacctgcagagcttctcaggacgtgaataccgctgtggcgtggtaccagcagaagccaggcaaagcgcctaagcttctcatttatagtgccagcttcctgtactcaggtgttccgtctcgcttttctggaagtagaagtgggaccgatttcacattgacgatcagcagcttgcagcccgaagatttcgccacctactactgtcagcagcactacactaccccaccgacatttggtcaaggcacaaaagtagagattaaacgcactggttccaccagcgggagcgggaaacccggctctggggaggggagcgaggtccagctggtggaatccgggggtggtcttgtgcagccaggaggatccttgaggttgtcctgcgccgcaagcggctttaacatcaaagatacatacatccattgggtccgacaggcccctggaaagggcctggagtgggtcgcccggatctacccaactaacgggtacactcgctacgctgatagcgtcaagggtcggtttactatttctgccgacacctcaaaaaacacagcctacctccagatgaactctctcagagctgaggatacagccgtgtactattgcagccggtggggaggcgacgggttctacgctatggatgtgtgggggcagggcacactggtcaccgtgagctcatccggaaccacgacgccagcgccgcgaccaccaacaccggcgcccaccatcgcgtcgcagcccctgtccctgcgcccagaggcgtgccggccagcggcggggggcgcagtgcacacgagggggctggacttcgcctgtgatatctacatctgggcgcccttggccgggacttgtggggtccttctcctgtcactggttatcaccctttactgcaaacggggcagaaagaaactcctgtatatattcaaacaaccatttatgagaccagtacaaactactcaagaggaagatggctgtagctgccgatttccagaagaagaagaaggaggatgtgaactgagagtgaagttcagcaggagcgcagacgcccccgcgtacaagcagggccagaaccagctctataacgagctcaatctaggacgaagagaggagtacgatgttttggacaagagacgtggccgggaccctgagatggggggaaagccgagaaggaagaaccctcaggaaggcctgtacaatgaactgcagaaagataagatggcggaggcctacagtgagattgggatgaaaggcgagcgccggaggggcaaggggcacgatggcctttaccagggtctcagtacagccaccaaggacacctacgacgcccttcacatgcaggccctgccccctcgctaag

SEQ ID NO: 19 - DNA, 3692 bp, synthetic construct
  misc_feature 1..3692: note = pASP31
  source 1..3692: mol_type = other DNA
tcgagttaattaagctagcttacttgtacagctcgtccatgccgagagtgatcccggcggcggtcacgaactccagcaggaccatgtgatcgcgcttctcgttggggtctttgctcagggcggactgggtgctcaggtagtggttgtcgggcagcagcacggggccgtcgccgatgggggtgttctgctggtagtggtcggcgagctgcacgctgccgtcctcgatgttgtggcggatcttgaagttcaccttgatgccgttcttctgcttgtcggccatgatatagacgttgtggctgttgtagttgtactccagcttgtgccccaggatgttgccgtcctccttgaagtcgatgcccttcagctcgatgcggttcaccagggtgtcgccctcgaacttcacctcggcgcgggtcttgtagttgccgtcgtccttgaagaagatggtgcgctcctggacgtagccttcgggcatggcggacttgaagaagtcgtgctgcttcatgtggtcggggtagcggctgaagcactgcacgccgtaggtcagggtggtcacgagggtgggccagggcacgggcagcttgccggtggtgcagatgaacttcagggtcagcttgccgtaggtggcatcgccctcgccctcgccggacacgctgaacttgtggccgtttacgtcgccgtccagctcgaccaggatgggcaccaccccggtgaacagctcctcgcccttgctcaccatggtggctttaccaacagtaccggaatgcccccgggctggaagtcgagcttccattatataccctctaactagtacgccttctgtatgaaacagtttttcctccacgccttctgtatgaaacagtttttcctccacgccttctgtatgaaacagtttttcctccacgccttctgtatgaaacagtttttcctccacgccttctgtatgaaacagtttttcctccacgccttctgtatgaaacagtttttcctccaacagtaccggatgcatcgtgaggctccggtgcccgtcagtgggcagagcgcacatcgcccacagtccccgagaagttggggggaggggtcggcaattgaaccggtgcctagagaaggtggcgcggggtaaactgggaaagtgatgtcgtgtactggctccgcctttttcccgagggtgggggagaaccgtatataagtgcagtagtcgccgtgaacgttctttttcgcaacgggtttgccgccagaacacaggtaagtgccgtgtgtggttcccgcgggcctggcctctttacgggttatggcccttgcgtgccttgaattacttccacctggctgcagtacgtgattcttgatcccgagcttcgggttggaagtgggtgggagagttcgaggccttgcgcttaaggagccccttcgcctcgtgcttgagttgaggcctggcctgggcgctggggccgccgcgtgcgaatctggtggcaccttcgcgcctgtctcgctgctttcgataagtctctagccatttaaaatttttgatgacctgctgcgacgctttttttctggcaagatagtcttgtaaatgcgggccaagatctgcacactggtatttcggtttttggggccgcgggcggcgacggggcccgtgcgtcccagcgcacatgttcggcgaggcggggcctgcgagcgcggccaccgagaatcggacgggggtagtctcaagctggccggcctgctctggtgcctggcctcgcgccgccgtgtatcgccccgccctgggcggcaaggctggcccggtcggcaccagttgcgtgagcggaaagatggccgcttcccggccctgctgcagggagctcaaaatggaggacgcggcgctcgggagagcgggcgggtgagtcacccacacaaaggaaaagggcctttccgtcctcagccgtcgcttcatgtgactccactgagtaccgggcgccgtccaggcacctcgattagttctcgtgcttttggagtacgtcgtctttaggttggggggaggggttttatgcgatggagtttccccacactgagtgggtggagactgaagttaggccagcttggcacttgatgtaattctccttggaatttgccctttttgagtttggatcttggttcattctcaagcctcagacagtggttcaaagtttttttcttccatttcaggtgtcgtgattctagagccaccatggccttaccagtgaccgccttgctcctgccgctggccttgctgctccacgccgccaggccggacattcaaatgacacagagtccctcatccctcagtgccagcgtgggcgatcgggtgactataacctgcagagcttctcaggacgtgaataccgctgtggcgtggtaccagcagaagccaggcaaagcgcctaagcttctcatttatagtgccagcttcctgtactcaggtgttccgtctcgcttttctggaagtagaagtgggaccgatttcacattgacgatcagcagcttgcagcccgaagatttcgccacctactactgtcagcagcactacactaccccaccgacatttggtcaaggcacaaaagtagagattaaacgcactggttccaccagcgggagcgggaaacccggctctggggaggggagcgaggtccagctggtggaatccgggggtggtcttgtgcagccaggaggatccttgaggttgtcctgcgccgcaagcggctttaacatcaaagatacatacatccattgggtccgacaggcccctggaaagggcctggagtgggtcgcccggatctacccaactaacgggtacactcgctacgctgatagcgtcaagggtcggtttactatttctgccgacacctcaaaaaacacagcctacctccagatgaactctctcagagctgaggatacagccgtgtactattgcagccggtggggaggcgacgggttctacgctatggatgtgtgggggcagggcacactggtcaccgtgagctcatccggaaccacgacgccagcgccgcgaccaccaacaccggcgcccaccatcgcgtcgcagcccctgtccctgcgcccagaggcgtgccggccagcggcggggggcgcagtgcacacgagggggctggacttcgcctgtgatttttgggtgctggtggtggttggtggagtcctggcttgctatagcttgctagtaacagtggcctttattattttctgggtgaggagtaagaggagcaggctcctgcacagtgactacatgaacatgactccccgccgccccgggcccacccgcaagcattaccagccctatgccccaccacgcgacttcgcagcctatcgctccatcgatagagtgaagttcagcaggagcgcagacgcccccgcgtaccagcagggccagaaccagctctataacgagctcaatctaggacgaagagaggagtacgatgttttggacaagagacgtggccgggaccctgagatggggggaaagccgagaaggaagaaccctcaggaaggcctgtacaatgaactgcagaaagataagatggcggaggcctacagtgagattgggatgaaaggcgagcgccggaggggcaaggggcacgatggcctttaccagggtctcagtacagccaccaaggacacctacgacgcccttcacatgcaggccctgccccctcgctaag

SEQ ID NO: 20 - DNA, 4559 bp, synthetic construct
  misc_feature 1..4559: note = pASP38
  source 1..4559: mol_type = other DNA
tcgagttaattaagctagcccggtactgttggaggaaaaactgtttcatacagaaggcgtggaggaaaaactgtttcatacagaaggcgtggaggaaaaactgtttcatacagaaggcgtggaggaaaaactgtttcatacagaaggcgtggaggaaaaactgtttcatacagaaggcgtggaggaaaaactgtttcatacagaaggcgtactagttagagggtatataatggaagctcgacttccagcccgggggcattccggtactgttggtaaagccaccatgtgccaccagcagctggtcatcagctggttcagcctggtgttcctggccagccctctggtggccatctgggagctgaagaaagacgtgtacgtggtggaactggactggtatcccgacgcccctggcgagatggtggtgctgacctgcgacacccctgaagaggacggcatcacctggaccctggaccagtctagcgaggtgctgggcagcggcaagaccctgaccatccaggtcaaagagttcggcgacgccggccagtacacctgtcacaagggcggagaggtgctgagccacagcctgctgctgctccacaagaaagaggatggcatttggagcaccgacatcctgaaggaccagaaagagcccaagaacaagaccttcctgagatgcgaggccaagaactacagcggccggttcacctgttggtggctgaccaccatcagcaccgacctgaccttcagcgtgaagtccagcagaggcagcagcgaccctcagggcgtgacatgtggcgccgctacactgtctgccgagagagtgcggggcgacaacaaagagtacgagtacagcgtcgagtgccaggaagatagcgcctgccctgccgccgaggaaagcctgcctatcgaagtgatggtggacgccgtgcacaagctgaagtacgagaactacacctccagctttttcatccgggacatcatcaagcccgaccctcccaagaacctgcagctgaagcctctgaagaacagcagacaggtggaagtgtcctgggagtaccccgacacctggtccacccctcacagctacttcagcctgacattctgtgtgcaagtccagggcaagtccaagcgcgagaaaaaggaccgggtgttcaccgacaagaccagcgccaccgtgatctgccggaagaacgcctctatcagcgtgcgggcccaggaccggtactacagcagctcttggagcgagtgggccagcgtgccatgttctggtggcggaggcggcggaagcagaaatctgccagtggccacccctgaccccggcatgtttccttgtctgcaccacagccagaacctgctgcgggccgtgtccaacatgctgcagaaggcccggcagaccctggaattctacccctgcaccagcgaggaaatcgaccacgaggacatcaccaaggataagaccagcaccgtggaagcctgtctgcccctggaactgaccaagaacgagagctgcctgaacagccgggaaaccagcttcatcaccaacggcagctgtctggccagcagaaagacctccttcatgatggccctgtgcctgagcagcatctacgaggacctgaagatgtaccaggtcgagttcaagaccatgaacgccaagctgctgatggaccccaagcggcagatctttctggaccagaatatgctggccgtgatcgacgagctgatgcaggccctgaacttcaacagcgagacagtgccccagaagtcctccctggaagaacccgacttctacaagaccaagatcaagctgtgcatcctgctgcacgccttccggatcagagccgtgaccatcgacagagtgatgagctacctgaacgcctcctaaatgcatcgtgaggctccggtgcccgtcagtgggcagagcgcacatcgcccacagtccccgagaagttggggggaggggtcggcaattgaaccggtgcctagagaaggtggcgcggggtaaactgggaaagtgatgtcgtgtactggctccgcctttttcccgagggtgggggagaaccgtatataagtgcagtagtcgccgtgaacgttctttttcgcaacgggtttgccgccagaacacaggtaagtgccgtgtgtggttcccgcgggcctggcctctttacgggttatggcccttgcgtgccttgaattacttccacctggctgcagtacgtgattcttgatcccgagcttcgggttggaagtgggtgggagagttcgaggccttgcgcttaaggagccccttcgcctcgtgcttgagttgaggcctggcctgggcgctggggccgccgcgtgcgaatctggtggcaccttcgcgcctgtctcgctgctttcgataagtctctagccatttaaaatttttgatgacctgctgcgacgctttttttctggcaagatagtcttgtaaatgcgggccaagatctgcacactggtatttcggtttttggggccgcgggcggcgacggggcccgtgcgtcccagcgcacatgttcggcgaggcggggcctgcgagcgcggccaccgagaatcggacgggggtagtctcaagctggccggcctgctctggtgcctggcctcgcgccgccgtgtatcgccccgccctgggcggcaaggctggcccggtcggcaccagttgcgtgagcggaaagatggccgcttcccggccctgctgcagggagctcaaaatggaggacgcggcgctcgggagagcgggcgggtgagtcacccacacaaaggaaaagggcctttccgtcctcagccgtcgcttcatgtgactccactgagtaccgggcgccgtccaggcacctcgattagttctcgtgcttttggagtacgtcgtctttaggttggggggaggggttttatgcgatggagtttccccacactgagtgggtggagactgaagttaggccagcttggcacttgatgtaattctccttggaatttgccctttttgagtttggatcttggttcattctcaagcctcagacagtggttcaaagtttttttcttccatttcaggtgtcgtgattctagagccaccatggccttaccagtgaccgccttgctcctgccgctggccttgctgctccacgccgccaggccggacattcaaatgacacagagtccctcatccctcagtgccagcgtgggcgatcgggtgactataacctgcagagcttctcaggacgtgaataccgctgtggcgtggtaccagcagaagccaggcaaagcgcctaagcttctcatttatagtgccagcttcctgtactcaggtgttccgtctcgcttttctggaagtagaagtgggaccgatttcacattgacgatcagcagcttgcagcccgaagatttcgccacctactactgtcagcagcactacactaccccaccgacatttggtcaaggcacaaaagtagagattaaacgcactggttccaccagcgggagcgggaaacccggctctggggaggggagcgaggtccagctggtggaatccgggggtggtcttgtgcagccaggaggatccttgaggttgtcctgcgccgcaagcggctttaacatcaaagatacatacatccattgggtccgacaggcccctggaaagggcctggagtgggtcgcccggatctacccaactaacgggtacactcgctacgctgatagcgtcaagggtcggtttactatttctgccgacacctcaaaaaacacagcctacctccagatgaactctctcagagctgaggatacagccgtgtactattgcagccggtggggaggcgacgggttctacgctatggatgtgtgggggcagggcacactggtcaccgtgagctcatccggaaccacgacgccagcgccgcgaccaccaacaccggcgcccaccatcgcgtcgcagcccctgtccctgcgcccagaggcgtgccggccagcggcggggggcgcagtgcacacgagggggctggacttcgcctgtgatatctacatctgggcgcccttggccgggacttgtggggtccttctcctgtcactggttatcaccctttactgcaaacggggcagaaagaaactcctgtatatattcaaacaaccatttatgagaccagtacaaactactcaagaggaagatggctgtagctgccgatttccagaagaagaagaaggaggatgtgaactgagagtgaagttcagcaggagcgcagacgcccccgcgtacaagcagggccagaaccagctctataacgagctcaatctaggacgaagagaggagtacgatgttttggacaagagacgtggccgggaccctgagatggggggaaagccgagaaggaagaaccctcaggaaggcctgtacaatgaactgcagaaagataagatggcggaggcctacagtgagattgggatgaaaggcgagcgccggaggggcaaggggcacgatggcctttaccagggtctcagtacagccaccaaggacacctacgacgcccttcacatgcaggccctgccccctcgctaag

SEQ ID NO: 21 - DNA, 4505 bp, synthetic construct
  misc_feature 1..4505: note = pASP52
  source 1..4505: mol_type = other DNA
tcgagttaattaagctagcttacatatgtctcttggcccgcaggtcctcttcggagatcagcttctgctcgcttcccttgccaggagacaggctcagggacttctgggtgtagtggttgtgcagggcctcgtgcatcacgctgcaggagaacacgtttccctgctgccatctgctcttgtccactgtcagcttgctgtacaggaagaatgagccgtcgctgtccagcacaggaggggttgtcttgtagttgttctcaggctggccattgctctcccattccacggcaatgtcgctggggtaaaagcccttgaccaggcaggtcagggacacctgattcttggtcagctcgtccctgcttggaggcagtgtgtaaacctggggttccctaggctggcccttggccttgctgatggttttctcgataggagcaggcagggccttgttggacaccttgcacttgtactctttgccgttcagccaatcctggtgcagcacggtcagcacggacaccactctgtaggtgctgttgtactgttcctctctaggcttggtcttggcgttgtgcacttccacgccgtccacgtaccaattgaacttcacttcggggtcctcgtgagacacatccaccaccacgcaggtcacttcaggggttctgctgatcatcagggtgtccttaggctttggaggaaacaggaacacggaaggtccgccgagcagttctggagcaggacatggaggacaggtgtgggtcttgtcgctgctcttgggttccactttgatttccaccttggtgccctggccaaatgtgtaaggcagggtgttgccctgctggcagtagtaggtggcaatgtcctcaggctgcaggctagatatggtgaaggtgaagtcggtgccgctgccagagccagaaaatctgctgggcacgccgctgtgcagtctgctggtgtagtagatcagcagtttaggggccttgccgggcttttgctgataccaattcaggtagctgctgatgtcctggctggcccgacaggtgattgtcactctgtctcccacagaggcagacaggctgctggggctctgtgtcatctgaatatcgctaccgcctccgccacttcctccgccaccagatcctccgcctccgctagaaacggtgaccagagagccctggccccaataatccatggcggtggttctggccaggcttctggcgcagtagtacacggctgtatcagcagcggtcacgctagacagccgcaggctgaactggttcttgctggtgtctctcagcatggtcactctggacttcaggctgggattgtaggtggtgatgccgctgtagctgatgtagccgatccattccaggcctcttccaggaggttgtcggacccaggaccaggcatgatcgctggtgatgctgtagccggacacggtacaggtcaggctcagtgtttggctaggccgcacgagtccaggtccagactcttgcagctgaacctcgcactgcacgcctctaagcagagccaccaggaacacccagctcaggccgaattccatggtggctttaccaacagtaccggaatgcccccgggctggaagtcgagcttccattatataccctctaactagtacgccttctgtatgaaacagtttttcctccacgccttctgtatgaaacagtttttcctccacgccttctgtatgaaacagtttttcctccacgccttctgtatgaaacagtttttcctccacgccttctgtatgaaacagtttttcctccacgccttctgtatgaaacagtttttcctccaacagtaccggatgcatcgtgaggctccggtgcccgtcagtgggcagagcgcacatcgcccacagtccccgagaagttggggggaggggtcggcaattgaaccggtgcctagagaaggtggcgcggggtaaactgggaaagtgatgtcgtgtactggctccgcctttttcccgagggtgggggagaaccgtatataagtgcagtagtcgccgtgaacgttctttttcgcaacgggtttgccgccagaacacaggtaagtgccgtgtgtggttcccgcgggcctggcctctttacgggttatggcccttgcgtgccttgaattacttccacctggctgcagtacgtgattcttgatcccgagcttcgggttggaagtgggtgggagagttcgaggccttgcgcttaaggagccccttcgcctcgtgcttgagttgaggcctggcctgggcgctggggccgccgcgtgcgaatctggtggcaccttcgcgcctgtctcgctgctttcgataagtctctagccatttaaaatttttgatgacctgctgcgacgctttttttctggcaagatagtcttgtaaatgcgggccaagatctgcacactggtatttcggtttttggggccgcgggcggcgacggggcccgtgcgtcccagcgcacatgttcggcgaggcggggcctgcgagcgcggccaccgagaatcggacgggggtagtctcaagctggccggcctgctctggtgcctggcctcgcgccgccgtgtatcgccccgccctgggcggcaaggctggcccggtcggcaccagttgcgtgagcggaaagatggccgcttcccggccctgctgcagggagctcaaaatggaggacgcggcgctcgggagagcgggcgggtgagtcacccacacaaaggaaaagggcctttccgtcctcagccgtcgcttcatgtgactccactgagtaccgggcgccgtccaggcacctcgattagttctcgtgcttttggagtacgtcgtctttaggttggggggaggggttttatgcgatggagtttccccacactgagtgggtggagactgaagttaggccagcttggcacttgatgtaattctccttggaatttgccctttttgagtttggatcttggttcattctcaagcctcagacagtggttcaaagtttttttcttccatttcaggtgtcgtgattctagaatggccttaccagtgaccgccttgctcctgccgctggccttgctgctccacgccgccaggccgggatccgacatcgttctgagtcagagccccgccatactgagcgcctcccccggggagaaggtgaccatgacctgtagagccagctccagcctttcatttatgcactggtaccagcagaaacccggtagtagtccaaagccgtggatttacgctacatccaacctggcaagcggagtaccagcccgcttctccggcagcggatcaggaacctcctactccctgacaatcagccgcgtcgaagccgaggatgcagccacatacttttgccaccagtggtcctctaatcccctgacatttggcgcaggcaccaagctcgaactgaagcggggatctaccagcggcagtggaaaacctggtagcggagaggggtctaccaaggggcaagtgcaactcagacagcctggcgcagaactcgtgaagcccggcgcatccgtcaagatgtcttgtaaagccagtggctacaccttcactagctataatatgcactgggttaaacagactcccggtcagggcctcgagtggattggcgcaatctacccgggtaatggtgatacttcttacaatcagaagtttaaggggaaagctaccctgaccgccgacaagtcttcatcaaccgcctacatgcagctgagctctctgacgtctgaggattccgccgtgtattactgcgcccggagccactacgggagtaattatgtcgattattttgactactggggtcagggaacaaccctgactgtctccagctccggaaccacgacgccagcgccgcgaccaccaacaccggcgcccaccatcgcgtcgcagcccctgtccctgcgcccagaggcgtgccggccagcggcggggggcgcagtgcacacgagggggctggacttcgcctgtgatatctacatctgggcgcccttggccgggacttgtggggtccttctcctgtcactggttatcaccctttactgcaaacggggcagaaagaaactcctgtatatattcaaacaaccatttatgagaccagtacaaactactcaagaggaagatggctgtagctgccgatttccagaagaagaagaaggaggatgtgaactgagagtgaagttcagcaggagcgcagacgcccccgcgtacaagcagggccagaaccagctctataacgagctcaatctaggacgaagagaggagtacgatgttttggacaagagacgtggccgggaccctgagatggggggaaagccgagaaggaagaaccctcaggaaggcctgtacaatgaactgcagaaagataagatggcggaggcctacagtgagattgggatgaaaggcgagcgccggaggggcaaggggcacgatggcctttaccagggtctcagtacagccaccaaggacacctacgacgcccttcacatgcaggccctgccccctcgctaag

SEQ ID NO: 22 - protein, 509 aa, synthetic construct
  REGION 1..509: note = anti-hIL-6R scFv-Fc
MEFGLSWVFLVALLRGVQCEVQLQESGPGLVRPSQTLSLTCTVSGYSITSDHAWSWVRQPPGRGLEWIGYISYSGITTYNPSLKSRVTMLRDTSKNQFSLRLSSVTAADTAVYYCARSLARTTAMDYWGQGSLVTVSSGGGGSGGGGSGGGGSDIQMTQSPSSLSASVGDRVTITCRASQDISSYLNWYQQKPGKAPKLLIYYTSRLHSGVPSRFSGSGSGTDFTFTISSLQPEDIATYYCQQGNTLPYTFGQGTKVEIKVEPKSSDKTHTCPPCPAPELLGGPSVFLFPPKPKDTLMISRTPEVTCVVVDVSHEDPEVKFNWYVDGVEVHNAKTKPREEQYNSTYRVVSVLTVLHQDWLNGKEYKCKVSNKALPAPIEKTISKAKGQPREPQVYTLPPSRDELTKNQVSLTCLVKGFYPSDIAVEWESNGQPENNYKTTPPVLDSDGSFFLYSKLTVDKSRWQQGNVFSCSVMHEALHNHYTQKSLSLSPGKGSEQKLISEEDLRAKR

SEQ ID NO: 23 - protein, 495 aa, synthetic construct
  REGION 1..495: note = Anti-CD20 CAR human
MALPVTALLLPLALLLHAARPGSDIVLSQSPAILSASPGEKVTMTCRASSSLSFMHWYQQKPGSSPKPWIYATSNLASGVPARFSGSGSGTSYSLTISRVEAEDAATYFCHQWSSNPLTFGAGTKLELKRGSTSGSGKPGSGEGSTKGQVQLRQPGAELVKPGASVKMSCKASGYTFTSYNMHWVKQTPGQGLEWIGAIYPGNGDTSYNQKFKGKATLTADKSSSTAYMQLSSLTSEDSAVYYCARSHYGSNYVDYFDYWGQGTTLTVSSSGTTTPAPRPPTPAPTIASQPLSLRPEACRPAAGGAVHTRGLDFACDIYIWAPLAGTCGVLLLSLVITLYCKRGRKKLLYIFKQPFMRPVQTTQEEDGCSCRFPEEEEGGCELRVKFSRSADAPAYKQGQNQLYNELNLGRREEYDVLDKRRGRDPEMGGKPRRKNPQEGLYNELQKDKMAEAYSEIGMKGERRRGKGHDGLYQGLSTATKDTYDALHMQALPPR

SEQ ID NO: 24 - protein, 495 aa, synthetic construct
  REGION 1..495: note = Anti-CD20 CAR canine
MASRVTALLLPLALLLRAAAASDIVLSQSPAILSASPGEKVTMTCRASSSLSFMHWYQQKPGSSPKPWIYATSNLASGVPARFSGSGSGTSYSLTISRVEAEDAATYFCHQWSSNPLTFGAGTKLELKRGSTSGSGKPGSGEGSTKGQVQLRQPGAELVKPGASVKMSCKASGYTFTSYNMHWVKQTPGQGLEWIGAIYPGNGDTSYNQKFKGKATLTADKSSSTAYMQLSSLTSEDSAVYYCARSHYGSNYVDYFDYWGQGTTLTVSSASPTTPAPRPPTRAPTNASKPVSPRGETCRPAAGSAVKTSGLDFACEIYIWAPLAGTCAVLLLSLVITIICHGRKKLLYLFKQPFMRPVQTAQEEDACSCRFPEEEEGECDLRAKFGRSAAAPEHQQGPNQLYNELNLRGREEYEVLDKRRGLDPEMGGKQRKRNPQEVVYNALQKDKMAEAYSEIGIKSENQRRRGKGHDGLYQGLSTATKDTYDALHMQALPPR

SEQ ID NO: 25 - protein, 490 aa, synthetic construct
  REGION 1..490: note = Anti-Her2 human CAR with 4-1BB costimulatory domain
MALPVTALLLPLALLLHAARPDIQMTQSPSSLSASVGDRVTITCRASQDVNTAVAWYQQKPGKAPKLLIYSASFLYSGVPSRFSGSRSGTDFTLTISSLQPEDFATYYCQQHYTTPPTFGQGTKVEIKRTGSTSGSGKPGSGEGSEVQLVESGGGLVQPGGSLRLSCAASGFNIKDTYIHWVRQAPGKGLEWVARIYPTNGYTRYADSVKGRFTISADTSKNTAYLQMNSLRAEDTAVYYCSRWGGDGFYAMDVWGQGTLVTVSSSGTTTPAPRPPTPAPTIASQPLSLRPEACRPAAGGAVHTRGLDFACDIYIWAPLAGTCGVLLLSLVITLYCKRGRKKLLYIFKQPFMRPVQTTQEEDGCSCRFPEEEEGGCELRVKFSRSADAPAYKQGQNQLYNELNLGRREEYDVLDKRRGRDPEMGGKPRRKNPQEGLYNELQKDKMAEAYSEIGMKGERRRGKGHDGLYQGLSTATKDTYDALHMQALPPR

SEQ ID NO: 26 - protein, 494 aa, synthetic construct
  REGION 1..494: note = Anti-Her2 CAR with CD28 costimulatory domain
MALPVTALLLPLALLLHAARPDIQMTQSPSSLSASVGDRVTITCRASQDVNTAVAWYQQKPGKAPKLLIYSASFLYSGVPSRFSGSRSGTDFTLTISSLQPEDFATYYCQQHYTTPPTFGQGTKVEIKRTGSTSGSGKPGSGEGSEVQLVESGGGLVQPGGSLRLSCAASGFNIKDTYIHWVRQAPGKGLEWVARIYPTNGYTRYADSVKGRFTISADTSKNTAYLQMNSLRAEDTAVYYCSRWGGDGFYAMDVWGQGTLVTVSSSGTTTPAPRPPTPAPTIASQPLSLRPEACRPAAGGAVHTRGLDFACDFWVLVVVGGVLACYSLLVTVAFIIFWVRSKRSRLLHSDYMNMTPRRPGPTRKHYQPYAPPRDFAAYRSIDRVKFSRSADAPAYQQGQNQLYNELNLGRREEYDVLDKRRGRDPEMGGKPRRKNPQEGLYNELQKDKMAEAYSEIGMKGERRRGKGHDGLYQGLSTATKDTYDALHMQALPPR

SEQ ID NO: 27 - protein, 532 aa, synthetic construct
  REGION 1..532: note = hIL-12 (p40-linker-p35)
MCHQQLVISWFSLVFLASPLVAIWELKKDVYVVELDWYPDAPGEMVVLTCDTPEEDGITWTLDQSSEVLGSGKTLTIQVKEFGDAGQYTCHKGGEVLSHSLLLLHKKEDGIWSTDILKDQKEPKNKTFLRCEAKNYSGRFTCWWLTTISTDLTFSVKSSRGSSDPQGVTCGAATLSAERVRGDNKEYEYSVECQEDSACPAAEESLPIEVMVDAVHKLKYENYTSSFFIRDIIKPDPPKNLQLKPLKNSRQVEVSWEYPDTWSTPHSYFSLTFCVQVQGKSKREKKDRVFTDKTSATVICRKNASISVRAQDRYYSSSWSEWASVPCSGGGGGGSRNLPVATPDPGMFPCLHHSQNLLRAVSNMLQKARQTLEFYPCTSEEIDHEDITKDKTSTVEACLPLELTKNESCLNSRETSFITNGSCLASRKTSFMMALCLSSIYEDLKMYQVEFKTMNAKLLMDPKRQIFLDQNMLAVIDELMQALNFNSETVPQKSSLEEPDFYKTKIKLCILLHAFRIRAVTIDRVMSYLNAS

SEQ ID NO: 28 - protein, 533 aa, synthetic construct
  REGION 1..533: note = cIL-12 (p40-linker-p35)
MHPQQLVISWFSLVLLASSLMTIWELEKDVYVVELDWHPDAPGEMVVLTCHTPEEDDITWTSAQSSEVLGSGKTLTIQVKEFGDAGQYTCHKGGKVLSRSLLLIHKKEDGIWSTDILKEQKESKNKIFLKCEAKNYSGRFTCWWLTAISTDLKFSVKSSRGFSDPQGVTCGAVTLSAERVRVDNRDYKKYTVECQEGSACPSAEESLPIEVVVDAIHKLKYENYTSSFFIRDIIKPDPPTNLQLKPLKNSRHVEVSWEYPDTWSTPHSYFSLTFCVQAQGKNNREKKDRLCVDKTSAKVVCHKDAKIRVQARDRYYSSSWSDWASVSCSGGGGGGSRSLPTASPSPGIFQCLNHSQNLLRAVSNTLQKARQTLELYSCTSEEIDHEDITKDKTSTVEACLPLELTMNESCLASREISLITNGSCLASGKASFMTVLCLSSIYEDLKMYQMEFKAMNAKLLMDPKRQIFLDQNMLTAIDELLQALNFNSVTVPQKSSLEEPDFYKTKIKLCILLHAFRIRAVTIDRMMSYLNSS

SEQ ID NO: 29 - DNA, 23 bp, synthetic construct
  misc_feature 1..23: note = Spacer
  source 1..23: mol_type = other DNA
ggcattccggtactgttggtaaa

SEQ ID NO: 30 - protein, 384 aa, Homo sapiens
MPQLDSGGGGAGGGDDLGAPDELLAFQDEGEEQDDKSRDSAAGPERDLAELKSSLVNESEGAAGGAGIPGVPGAGAGARGEAEALGREHAAQRLFPDKLPEPLEDGLKAPECTSGMYKETVYSAFNLLMHYPPPSGAGQHPQPQPPLHKANQPPHGVPQLSLYEHFNSPHPTPAPADISQKQVHRPLQTPDLSGFYSLTSGSMGQLPHTVSWFTHPSLMLGSGVPGHPAAIPHPAIVPPSGKQELQPFDRNLKTQAESKAEKEAKKPTIKKPLNAFMLYMKEMRAKVIAECTLKESAAINQILGRRWHALSREEQAKYYELARKERQLHMQLYPGWSARDNYGKKKRRSREKHQESTTETNWPRELKDGNGQESLSMSSSSSPA

SEQ ID NO: 31 - protein, 655 aa, Homo sapiens
MAEAPQVVEIDPDFEPLPRPRSCAWPLPRPEFSQSNSATSSPAPSGSAAANPDAAAGLPSASAAAVSADFMSNLSLLEESEDFPQAPGSVAAAVAAAAAAAATGGLCGDFQGPEAGCLHPAPPQPPPPGPLSQHPPVPPAAAGPLAGQPRKSSSSRRNAWGNLSYADLITKAIESSAEKRLTLSQIYEWMVKSVPYFKDKGDSNSSAGWKNSIRHNLSLHSKFIRVQNEGTGKSSWWMLNPEGGKSGKSPRRRAAAMDNNSKFAKSRSRAAKKKASLQSGQEGAGDSPGSQFSKWPASPGSHSNDDFDNWSTFRPRTSANASTISGRLSPIMTEQDDLGEGDVHSMVYPPSAAKMASTLPSLSEISNPENMENLLDNLNLLSSPTSLTVSTQSSPGTMMQQTPCYSFAPPNTSLNSPSPNYQKYTYGQSSMSPLPQMPIQTLQDNKSSYGGMSQYNCAPGLLKELLTSDSPPHNDIMTPVDPGVAQPNSRVLGQNVMMGPNSVMSTYGSQASHNKMMNPSSHTHPGHAQQTSAVNGRPLPHTVSTMPHTSGMNRLTQVKTPVQVPLPHPMQMSALGGYSSVSSCNGYGRMGLLHQEKLPSDLDGMFIERLDCDMESIIRNDLMDGDTLDFNFDNVLPNQSFPHSVKTTTHSWVSG

SEQ ID NO: 32 - DNA, 111 bp, synthetic construct
  misc_feature 1..111: note = STAT3 responsive element
  source 1..111: mol_type = other DNA
ccggtactgttagcttcatttcccgtaaatcgtcgaagcttcatttcccgtaaatcgtcgaagcttcatttcccgtaaatcgtcgaagcttcatttcccgtaaatcgtcga

SEQ ID NO: 33 - DNA, 1404 bp, synthetic construct
  misc_feature 1..1404: note = hIL-6Ra
  source 1..1404: mol_type = other DNA
atgctggccgtgggatgtgctttgcttgctgctctgttggctgctcctggtgctgcactggcccctagaagatgtcctgctcaagaggtggcaagaggcgtgctgacatctctgcctggcgatagcgtgaccctgacatgtcctggcgtggaacccgaggataatgccaccgtgcattgggtgctgagaaagcctgccgccggatctcatcctagcagatgggctggcatgggccgtagactgctgctgagatctgtccagctgcacgacagcggcaactacagctgttacagagccggcagacctgccggaacagtgcatctgctggtggatgtgcctcctgaggaaccccagctgagctgcttcagaaagtcccctctgagcaacgtcgtgtgcgagtggggccctagaagcacacctagcctgacaacaaaggccgtgctgctcgtgcggaagttccagaattctcccgccgaggacttccaagagccttgccagtacagccaagagagccagaagttcagctgtcagctggctgtgcctgagggcgacagcagcttctacatcgtgtctatgtgcgtggccagcagcgtgggcagcaagtttagcaagacccagaccttccaaggctgcggcatcctgcaacctgatcctccagccaacatcaccgtgaccgccgtggccagaaatcccagatggctgtctgtgacctggcaggaccctcacagctggaactccagcttttaccggctgagattcgagctgcggtacagggccgagagaagcaagaccttcaccacctggatggtcaaggacctgcagcatcactgcgtgatccacgatgcttggagcggcctgagacatgtggtgcagctgagagcccaagaggaattcggccaaggcgagtggagtgaatggtcccctgaagccatgggcaccccttggacagagagcagatctccaccagccgagaacgaggtgtccacacctatgcaggccctgaccaccaacaaggacgacgacaacatcctgttccgggacagcgccaatgccacaagtctgcctgtgcaggatagctcctctgtgcccctgcctacctttctggttgctggcggatctctggcctttggcaccctgctgtgtatcgccatcgtgctgcggttcaagaaaacctggaagctgcgggccctgaaagagggcaagacctctatgcaccctccttacagcctgggccagctggtgcctgaaagacctagacctacacctgtgctggtgcccctgatcagccctcctgtgtctccatctagcctgggcagcgacaataccagcagccacaacagacccgacgctcgggaccctagatctccctacgacatcagcaataccgactacttcttcccacgc

SEQ ID NO: 34 - DNA, 1422 bp, synthetic construct
  misc_feature 1..1422: note = Regulatory unit
  source 1..1422: mol_type = other DNA
aggctggatcggtcccggtgtcttctatggaggtcaaaacagcgtggatggcgtctccaggcgatctgacggttcactaaacgagctctgcttatataggcctcccaccgtacacgcctacggaggacagtactccgtgcggaggacagtactccgtccggaggacagtactccgatcggaggacagtactccggtcggaggacagtactccgctcggaggacagtactccgacgcgtcgtgaggctccggtgcccgtcagtgggcagagcgcacatcgcccacagtccccgagaagttggggggaggggtcggcaattgaaccggtgcctagagaaggtggcgcggggtaaactgggaaagtgatgtcgtgtactggctccgcctttttcccgagggtgggggagaaccgtatataagtgcagtagtcgccgtgaacgttctttttcgcaacgggtttgccgccagaacacaggtaagtgccgtgtgtggttcccgcgggcctggcctctttacgggttatggcccttgcgtgccttgaattacttccacctggctgcagtacgtgattcttgatcccgagcttcgggttggaagtgggtgggagagttcgaggccttgcgcttaaggagccccttcgcctcgtgcttgagttgaggcctggcctgggcgctggggccgccgcgtgcgaatctggtggcaccttcgcgcctgtctcgctgctttcgataagtctctagccatttaaaatttttgatgacctgctgcgacgctttttttctggcaagatagtcttgtaaatgcgggccaagatctgcacactggtatttcggtttttggggccgcgggcggcgacggggcccgtgcgtcccagcgcacatgttcggcgaggcggggcctgcgagcgcggccaccgagaatcggacgggggtagtctcaagctggccggcctgctctggtgcctggcctcgcgccgccgtgtatcgccccgccctgggcggcaaggctggcccggtcggcaccagttgcgtgagcggaaagatggccgcttcccggccctgctgcagggagctcaaaatggaggacgcggcgctcgggagagcgggcgggtgagtcacccacacaaaggaaaagggcctttccgtcctcagccgtcgcttcatgtgactccactgagtaccgggcgccgtccaggcacctcgattagttctcgtgcttttggagtacgtcgtctttaggttggggggaggggttttatgcgatggagtttccccacactgagtgggtggagactgaagttaggccagcttggcacttgatgtaattctccttggaatttgccctttttgagtttggatcttggttcattctcaagcctcagacagtggttcaaagtttttttcttccatttcaggtgtcgtga

SEQ ID NO: 35 - protein, 236 aa, synthetic construct
  REGION 1..236: note = mCherry reporter
MVSKGEEDNMAIIKEFMRFKVHMEGSVNGHEFEIEGEGEGRPYEGTQTAKLKVTKGGPLPFAWDILSPQFMYGSKAYVKHPADIPDYLKLSFPEGFKWERVMNFEDGGVVTVTQDSSLQDGEFIYKVKLRGTNFPSDGPVMQKKTMGWEASSERMYPEDGALKGEIKQRLKLKDGGHYDAEVKTTYKAKKPVQLPGAYNVNIKLDITSHNEDYTIVEQYERAEGRHSTGGMDELYK

SEQ ID NO: 36 - protein, 781 aa, synthetic construct
  REGION 1..781: note = 4D5-Notch1-Gal4-VP64 receptor
DIQMTQSPSSLSASVGDRVTITCRASQDVNTAVAWYQQKPGKAPKLLIYSASFLYSGVPSRFSGSRSGTDFTLTISSLQPEDFATYYCQQHYTTPPTFGQGTKVEIKRTGSTSGSGKPGSGEGSEVQLVESGGGLVQPGGSLRLSCAASGFNIKDTYIHWVRQAPGKGLEWVARIYPTNGYTRYADSVKGRFTISADTSKNTAYLQMNSLRAEDTAVYYCSRWGGDGFYAMDVWGQGTLVTVSSILDYSFTGGAGRDIPPPQIEEACELPECQVDAGNKVCNLQCNNHACGWDGGDCSLNFNDPWKNCTQSLQCWKYFSDGHCDSQCNSAGCLFDGFDCQLTEGQCNPLYDQYCKDHFSDGHCDQGCNSAECEWDGLDCAEHVPERLAAGTLVLVVLLPPDQLRNNSFHFLRELSHVLHTNVVFKRDAQGQQMIFPYYGHEEELRKHPIKRSTVGWATSSLLPGTSGGRQRRELDPMDIRGSIVYLEIDNRQCVQSSSQCFQSATDVAAFLGALASLGSLNIPYKIEAVKSEPVEPPLPSQLHLMYVAAAAFVLLFFVGCGVLLSRKRRRMKLLSSIEQACDICRLKKLKCSKEKPKCAKCLKNNWECRYSPKTKRSPLTRAHLTEVESRLERLEQLFLLIFPREDLDMILKMDSLQDIKALLTGLFVQDNVNKDAVTDRLASVETDMPLTLRQHRISATSSSEESSNKGQRQLTVSAAAGGSGGSGGSDALDDFDLDMLGSDALDDFDLDMLGSDALDDFDLDMLGSDALDDFDLDMLGS

SEQ ID NO: 37 - protein, 233 aa, synthetic construct
  REGION 1..233: note = BFP2 reporter
MSELIKENMHMKLYMEGTVDNHHFKCTSEGEGKPYEGTQTMRIKVVEGGPLPFAFDILATSFLYGSKTFINHTQGIPDFFKQSFPEGFTWERVTTYEDGGVLTATQDTSLQDGCLIYNVKIRGVNFTSNGPVMQKKTLGWEAFTETLYPADGGLEGRNDMALKLVGGSHLIANAKTTYRSKKPAKNLKMPGVYYVDYRLERIKEANNETYVEQHEVAVARYCDLPSKLGHKLN

SEQ ID NO: 38 - protein, 655 aa, Homo sapiens
MAEAPQVVEIDPDFEPLPRPRSCTWPLPRPEFSQSNSATSSPAPSGSAAANPDAAAGLPSASAAAVSADFMSNLSLLEESEDFPQAPGSVAAAVAAAAAAAATGGLCGDFQGPEAGCLHPAPPQPPPPGPLSQHPPVPPAAAGPLAGQPRKSSSSRRNAWGNLSYADLITKAIESSAEKRLTLSQIYEWMVKSVPYFKDKGDSNSSAGWKNSIRHNLSLHSKFIRVQNEGTGKSSWWMLNPEGGKSGKSPRRRAASMDNNSKFAKSRSRAAKKKASLQSGQEGAGDSPGSQFSKWPASPGSHSNDDFDNWSTFRPRTSSNASTISGRLSPIMTEQDDLGEGDVHSMVYPPSAAKMASTLPSLSEISNPENMENLLDNLNLLSSPTSLTVSTQSSPGTMMQQTPCYSFAPPNTSLNSPSPNYQKYTYGQSSMSPLPQMPIQTLQDNKSSYGGMSQYNCAPGLLKELLTSDSPPHNDIMTPVDPGVAQPNSRVLGQNVMMGPNSVMSTYGSQASHNKMMNPSSHTHPGHAQQTSAVNGRPLPHTVSTMPHTSGMNRLTQVKTPVQVPLPHPMQMSALGGYSSVSSCNGYGRMGLLHQEKLPSDLDGMFIERLDCDMESIIRNDLMDGDTLDFNFDNVLPNQSFPHSVKTTTHSWVSG

SEQ ID NO: 39 - DNA, 20 bp, synthetic construct
  misc_feature 1..20: note = TRAC
  source 1..20: mol_type = other DNA
tgtgctagacatgaggtcta

SEQ ID NO: 40 - DNA, 20 bp, synthetic construct
  misc_feature 1..20: note = TRBC
  source 1..20: mol_type = other DNA
ggagaatgacgagtggaccc